European Patent Application EP 4 653 525 A1, published November 26, 2025. Title: ENGINEERED TERMINAL DEOXYNUCLEOTIDYL TRANSFERASE POLYMERASES. Applicant: UAB Biomatter Designs. Application EP. The sequence listing filed with the application follows.

SEQUENCE LISTING (100 sequences)

SEQ ID NO: 1 - protein, 389 aa, Bos taurus
MGHQLVVRTDYSATPNPGFQKTPPLAVKKISQYACQRKTTLNNYNHIFTDAFEILAENSEFKENEVSYVTFMRAASVLKSLPFTIISMKDTEGIPCLGDKVKCIIEEIIEDGESSEVKAVLNDERYQSFKLFTSVFGVGLKTSEKWFRMGFRSLSKIMSDKTLKFTKMQKAGFLYYEDLVSCVTRAEAEAVGVLVKEAVWAFLPDAFVTMTGGFRRGKKIGHDVDFLITSPGSAEDEEQLLPKVINLWEKKGLLLYYDLVESTFEKFKLPSRQVDTLDHFQKCFLILKLHHQRVDSSKSNQQEGKTWKAIRVDLVMCPYENRAFALLGWTGSRQFERDIRRYATHERKMMLDNHALYDKTKRVFLKAESEEEIFAHLGLDYIEPWERNA

SEQ ID NO: 2 - protein, 389 aa, synthetic construct
MGHQLVVRTDYSATPNPGFQKTPPLAVKKISQYACQRKTTLDNKNKKFTDALEELAEYEEYKENEVSKVTFERAASVLKSLPFEIKSLKDLEGIPCLGDKIKKLIEEILENGYSKEVEKIKKDERYQTLKLFTSVFGVGLKTAKKWYRKGYRTLEEVKNDKTLKLTKMQKAGLKYYEDLTSGVTRAEAEAILVIVKEAVHAFLPDAEVTLVGGFRRGKKIGHDVDVLITSPGPAEDLEQLLPKVVNYLEEKGLLLYYDLVESTFEKFKLPSRQVDTLDHFAKCFMIIKLPHQWVDPSLSNQQEGKTWKAVRVDLVLAPYENRAFALLGWTGSRQFERDIRRYATHEKNMLLDNHGLYDKTKRVFLKAESEEEIFAHLGLDYVEPWERNA

SEQ ID NO: 3 - protein, 389 aa, synthetic construct
MGHQLVVRTDYSATPNPGFQKTPPLAVEKISQYACQRKTTLKNLNKKFTDAFEILAEYAEYKENEVSKVTFERAASVLKSLPFEIKSMEDTEGIPCLGDKIRKIIEEILEKGYSSEVEKVLKDERYQAFKLFTSVFGVGLKTAKKWYEKGYRTLEDIKKDKSLKFTKMQKAGFKYYEDLVAPVTRAEAEAVGKLVEEAVHEFLPDAKVTMVGGFRRGKKIGHDVDFLITTPGEEEKVKELLKKVIDLWEKKGLLLYYDLVESTFEKFKLPSRQVDTLDHFEKCFMILKLHYKEVDPSVSSHMEGKKWKAVRVDLVAAPYENYAFALLGWTGSRQFERDIRRYATHERNMLLDNHRLYDLTKREFLEAKSEEEIFEHLGLEYIEPHERNA

SEQ ID NO: 4 - protein, 389 aa, synthetic construct
MGHQLVVRTDYSATPNPGFQKTPPLAVEKISQYACQRKTTLKNLNKEFTDAFEILAEYAEYKENEVSKVTFERAASVLKSLPFKIESMEDTEGIPCLGDKIRKIIEEILEKGYSEEVRKVLEDERYQAFKLFTSVFGVGLKTAKKWYEKGYRTLEDIKKDKSLKFTKMQKAGFKYYEDLVAPVTRAEAEAVGKLVEEAVHEFLPDAKVTMVGGFRRGKKIGHDVDFLITTPGEEEKVKELLKKVIELWEKKGLLLYYDLVESTFEKFKLPSRQVDTLDHFEKCFMILKLPYELVDPSVSSHMEGKKWKAVRVDLVAAPYENYAFALLGWTGSRQFERDIRRYATHERNMLLDNHRLYDLTKREFLKAESEEEIFKHLGLEYIEPHERNA

SEQ ID NO: 5 - protein, 389 aa, synthetic construct
MGHQLVVRTDYSATPNPGFQKTPPLAVEKISQYACQRKTTLKNLNKEFTDAFEILAEYAEYKENEVSKVTFERAASVLKSLPFKIESMEDTEGIPCLGDKIRKIIEEILEKGYSEEVEKVLKDERYQAFKLFTSVFGVGLKTAKKWYEKGYRTLEDIKKDKSLKFTKMQKAGFKYYEDLVAPVTRAEAEAVGVLVKEAVHKFLPDAKVTMVGGFRRGKKIGHDVDFLITTPGEEEKVKELLKKVIDLWEKEGLLLYYDLVESTFEKFKLPSRQVDTLDHFEKCFLILKLDYKRVDPSVSSHMEGKKWKAVRVDLVAAPYENYAFALLGWTGSRQFERDIRRYATHERNMLLDNHRLYDLTERKFLEAKSEEEIFEHLGLEYIEPHERNA

SEQ ID NO: 6 - protein, 389 aa, synthetic construct
MGHQLVVRTDYSATPNPGFQKTPPLAVEKISQYACQRKTTLNNLNKEFTDAFEILAEDAEYKENEVSKVTFERAASVLKSLPFKIESMEDTEGIPCLGDKIRYIIEEILEKGYSSEVLEVLNDERYQAFKLFTSVFGVGLKTAKKWYEKGYRTLEDIKKDKSLKFTKMQKAGFKYYEDLVADVTRAEAEAVGVLVKEAVHKFLPDALVTMVGGFRRGKKIGHDVDFLITTPGDQEKLKELLKKVIDLWEKEGLLLYYDLVESTFEKFKLPSRQVDTLDHFEKCFLILKLHHVRVDPSKSLFMEGKKWKAVRVDLVAAPYENYAFALLGWTGSRQFERDIRRYATHERNMQLDNHRLYDETKREFLEAKSEEEIFEHLGLEYIEPHERNA

SEQ ID NO: 7 - protein, 389 aa, synthetic construct
MGHQLVVRTDYSATPNPGFQKTPPLAVKKISQYACQRKTTLKNLNKEFTDAFEILAEYAEYKENEVSKVTFERAASVLKSLPFKIESMEDTEGIPCLGDKIKKIIEEILEKGYSEEVKKVLEDERYQAFKLFTSVFGVGLKTAKKWYEKGYRTLEDIKKDKSLKFTKMQKAGFKYYEDLVAPVTRAEAEAVGVLVREAVHAFLPDAFVTMVGGFRRGKKIGHDVDFLITTPGSEEDRKTLLPKVINLWEKQGLLLYYDLVESTFEKFKLPSRQVDTLDHFEKCFCILKLHYQRVDPSVSNFQEGKTWKAVRVDLVLAPYENYAFALLGWTGSRQFERDIRRYATHERNMLLDNHRLYDLTKREFLKAESEEEIFAHLGLDYIEPWERNA

SEQ ID NO: 8 - protein, 389 aa, synthetic construct
MGHQLVVRTDYSATPNPGFQKTPPLAVKKISQYACQRKTTLDNKNKKFTDALEELAEYEEYKENEVSKVTFERAASVLKSLPFEIKSIKDLEGIPCLGDKIKKLIEEILENGYSKEVEKIKKDERYQTLKLFTSVFGVGLKTAKKWYRKGYRTLEEVKKDKTLKLTKMQKAGLKYYEDLTSGVTRAEAEAILVIVKEAVHAFLPDAEVTLVGGFRRGKKIGHDVDVLITSPGPAEDLEQLLPKVVNYLEEKGLLLYYDLVESTFEKFKLPSRQVDTLDHFAKCFMIIKLPHQWVDPSLSPQIEGKTWKAVRVDLVLAPYENRAFALLGWTGSRQFERDIRRYATHEKNMLLDNHRLYDKTKRVFLKAESEEEIFAHLGLDYVEPWERNA

SEQ ID NO: 9 - protein, 389 aa, synthetic construct
MGHQLVVRTDYSATPNPGFQKTPPLAVKKISQYACQRKTTLNNKNKKFTDALEILAEYEEYKENEVSKVTFERAASVLKSLPFEIKSIKDLEGIPCLGDKIKKLIEEILENGYSKEVEKIKKDERYQTLKLFTSVFGVGLKTAKKWYRKGYRTLEEVMKDKTLKFTKMQKAGFKYYEDLTSPVTRAEAEAIGVIVKEAVHAFLPDAEVTIVGGFRRGKKIGHDVDILITSPGPAEDLEQLLPKVVNYLEEKGLLLYYDLVESTFEKFKLPSRQVDTLDHFAKCFMIIKLPHQWVDPSLSNQQEGKTWKAVRVDLVLAPYENRAFALLGWTGSRQFERDIRRYATHEKNMLLDNHGLYDKTKRVFLKAESEEEIFAHLGLDYVEPWERNA

SEQ ID NO: 10 - protein, 389 aa, synthetic construct
MGHQLVVRTDYSATPNPGFQKTPPLAVKKISQYACQRKTTLNNYNKIFTDAFEILAENAEFKENEVSYVTFMRAASVLKSLPFTIKSMKDTEGIPCLGDKVKKIIEEIIEDGESSEVKAVLNDERYQSFKLFTSVFGVGLKTSEKWFRMGFRSLSEIKSDKTLKFTKMQKAGFLYYEDLVSCVTRAEAEAVGVLVKEAVHAFLPDAFVTITGGFRRGKKIGHDVDFLITSPGSPEDEEQLLPKVINLWEKKGLLLYSDLVESTFEKFKLPSRQVDTLDHFQKCFLILKLHHQRVDSSKSNQQEGKTWKAIRVDLVLCPYERRAFALLGWTGSRQFERDIRRYATHERKMLLDNHALYDKTKRVFLKAESEEEIFAHLGLDYIEPWERNA

SEQ ID NO: 11 - protein, 389 aa, synthetic construct
MGHQLVVRTDYSATPNPGFQKTPPLAVKKISQYACQRKTTLNNLNHIFTDAFEILAENAEYKENEVSYVTFMRAASVLKSLPFKIISMKDTEGIPCLGDKIKCIIEEILEDGESSEVKAVLNDERYQSFKLFTSVFGVGLKTAEKWYRMGYRSLSKIMSDKTLKFTKMQKAGFKYYEDLVAPVTRAEAEAVGVLVKEAVHAFLPDAFVTMVGGFRRGKKIGHDVDFLITSPGSAEDEEQLLPKVINLWEKKGLLLYYDLVESTFEKFKLPSRQVDTLDHFQKCFLILKLHHQRVDSSKSNQQEGKTWKAVRVDLVMCPYENRAFALLGWTGSRQFERDIRRYATHERNMLLDNHALYDKTKRVFLKAESEEEIFAHLGLDYIEPWERNA

SEQ ID NO: 12 - protein, 389 aa, synthetic construct
MGHQLVVRTDYSATPNPGFQKTPPLAVKKISQYACQRKTTLNNYNHIFTDAFEILAENAEFKENEVSYVTFMRAASVLKSLPFTIISMKDTEGIPCLGDKVKCIIEEIIEDGESSEVKAVLNDERYQSFKLFTSVFGVGLKTSEKWFRMGFRSLSEIMSDKTLKFTKMQKAGFLYYEDLVSCVTRAEAEAVGVLVKEAVHAFLPDAFVTMTGGFRRGKKIGHDVDFLITSPGSAEDEEQLLPKVINLWEKKGLLLYYDLVESTFEKFKLPSRQVDTLDHFQKCFLILKLHHQRVDSSKSNQQEGKTWKAIRVDLVLCPYENRAFALLGWTGSRQFERDIRRYATHERKMLLDNHALYDKTKRVFLKAESEEEIFAHLGLDYIEPWERNA

SEQ ID NO: 13 - protein, 389 aa, synthetic construct
MGHQLVVRTDYSATPNPGFQKTPPLAVKKISQYACQRKTTLNNYNKIFTDAFEILAENAEFKENEVSYVTFKRAASVLKSLPFTIKSMKDTEGIPCLGDKVKKIIEEIIEDGESSEVKAVLNDERYQSFKLFTSVFGVGLKTSEKWFRMGFRSLSEILSDKTLKFTKMQKAGFLYYEDLVSCVTRAEAEAVGELVKEAVHAFLPDAFVTITGGFRRGKKIGHDVDFLITSPGSEEDEEQLLPKVINLWEKKGLLLYSDLVESTFEKFKLPSRQVDTLDHFQKCFLILKLHHQRVDSSKSNQQEGKTWKAIRVDLVVCPYERRAFALLGWTGSRQFERDIRRYATHERKMLLDNHALYDKTKRVFLKAESEEEIFAHLGLDYIEPWERNA

SEQ ID NO: 14 - protein, 389 aa, synthetic construct
MGHQLVVRTDYSATPNPGFQKTPPLAVKKISQYACQRKTTLNNYNKIFTDAFEILAENAEFKENEVSYVTFMRAASVLKSLPFTIKSMKDTEGIPCLGDKVKKIIEEIIEDGESSEVKAVLNDERYQSFKLFTSVFGVGLKTSEKWFRMGFRSLSDIMSDKTLKFTKMQKAGFLYYEDLVSCVTRAEAEAVGVLVKEAVHAFLPDAFVTMTGGFRRGKKIGHDVDFLITSPGSAEDEEQLLPKVINLWEKKGLLLYYDLVESTFEKFKLPSRQVDTLDHFQKCFLILKLHHQRVDSSKSNQQEGKTWKAIRVDLVLCPYENRAFALLGWTGSRQFERDIRRYATHERKMLLDNHALYDKTKRVFLKAESEEEIFAHLGLDYIEPWERNA

SEQ ID NO: 15 - protein, 389 aa, synthetic construct
MGHQLVVRTDYSATPNPGFQKTPPLAVKKISQYACQRKTTLNNYNHIFTDAFEILAENAEYKENEVSYVTFMRAASVLKSLPFTIISMKDTEGIPCLGDKIKCIIEEILEDGESSEVKAVLNDERYQSFKLFTSVFGVGLKTAEKWYRMGYRSLSKIMSDKTLKFTKMQKAGFLYYEDLVSCVTRAEAEAVGVLVKEAVHAFLPDAFVTMTGGFRRGKKIGHDVDFLITSPGSAEDEEQLLPKVINLWEKKGLLLYYDLVESTFEKFKLPSRQVDTLDHFQKCFLILKLHHQRVDSSKSNQQEGKTWKAIRVDLVMCPYENRAFALLGWTGSRQFERDIRRYATHERKMLLDNHALYDKTKRVFLKAESEEEIFAHLGLDYIEPWERNA

SEQ ID NO: 16 - protein, 389 aa, synthetic construct
MGHQLVVRTDYSATPNPGFQKTPPLAVKKISQYACQRKTTLNNYNHIFTDAFEILAENYEFKENEVSYVTFMRAASVLKSLPFTIISMKDTEGLPCLGDKVKCIIEEIIEDGESSEVKAVLNDERYQSFKLFTSVFGVGLKTSEKWFRMGFRSLSKIMSDKTLKFTKMQKAGFLYYEDLVSCVTRAEAEAVGVLVKEAVWAFLPDAFVTMTGGFRRGKKIGHDVDFLITSPGSAEDEEQLLPKVINLWEKKGLLLYYDLVESTFEKFKLPSRQVDTLDHFQKCFLILKLHHQRVDSSKSNQQEGKTWKAIRVDLVMCPYENYAFALLGWTGSRQFERDLRRYATHERKMMLDNHALYDKTKRVFLKAESEEEIFAHLGLDYIEPWERNA

SEQ ID NO: 17 - protein, 389 aa, synthetic construct
MGHQLVVRTDYSATPNPGFQKTPPLAVKKISQYACQRKTTLNNYNHIFTDALEILAEYSEFKENEVSYVTFMRAASVLKSLPFTIISMKDTEGIPCLGDKVKCIIEEILEDGESSEVKAVLNDERYQSFKLFTSVFGVGLKTAEKWFRMGYRSLSKIMSDKTLKFTKMQKAGFLYYEDLVSCVTRAEAEAVGVLVKEAVWAFLPDAFVTMVGGFRRGKKIGHDVDFLITSPGSAEDLEQLLPKVINLLEKKGLLLYYDLVESTFEKFKLPSRQVDTLDHFQKCFLILKLHHQRVDSSKSNQQEGKTWKAVRVDLVMCPYENRAFALLGWTGSRQFERDIRRYATHERKMLLDNHALYDKTKRVFLKAESEEEIFAHLGLDYIEPWERNA

SEQ ID NO: 18 - protein, 389 aa, synthetic construct
MGHQLVVRTDYSATPNPGFQKTPPLAVKKISQYACQRKTTLNNYNHKFTDALEILAEYSEFKENEVSYVTFMRAASVLKSLPFTIISMKDTEGIPCLGDKIKCLIEEILEDGESSEVKAIKNDERYQTLKLFTSVFGVGLKTAKKWYRMGYRSLSKVMSDKTLKFTKMQKAGFLYYEDLVSPVTRAEAEAVGVIVKEAVWAFLPDAFVTMVGGFRRGKKIGHDVDFLITSPGSAEDLEQLLPKVINLLEKKGLLLYYDLVESTFEKFKLPSRQVDTLDHFQKCFLIIKLPHQWVDSSKSNQQEGKTWKAVRVDLVLAPYENRAFALLGWTGSRQFERDIRRYATHERKMLLDNHRLYDKTKRVFLKAESEEEIFAHLGLDYVEPWERNA

SEQ ID NO: 19 - protein, 389 aa, synthetic construct
MGHQLVVRTDYSATPNPGFQKTPPLAVKKISQYACQRKTTLNNKNHKFTDALEILAEYSEYKENEVSYVTFMRAASVLKSLPFTIISMKDLEGIPCLGDKIKCLIEEILENGYSSEVKAIKNDERYQTLKLFTSVFGVGLKTAKKWYRKGYRSLSELMSDKTLKFTKMQKAGFKYYEDLVSPVTRAEAEAIGVIVKEAVHAFLPDAEVTMVGGFRRGKKIGHDVDFLITSPGSAEDLEQLLPKVVNLLEEKGLLLYYDLVESTFEKFKLPSRQVDTLDHFAKCFMIIKLPHQWVDPSKSNQQEGKTWKAVRVDLVLAPYENRAFALLGWTGSRQFERDIRRYATHEKNMGLDNHRLYDKTKRVFLKAESEEEIFAHLGLDYVEPWERNA

SEQ ID NO: 20 - protein, 389 aa, synthetic construct
MGHQLVVRTDYSATPNPGFQKTPPLAVKPLSQYACQRRTTLQNNNKKFTDALEVLAEYEEYKENEVSKVTFERAASVLKSLPKEIKSLKDIEGIPCLGDKTKKIIEEILENGYSKEVEKIKKDERYQALKLFTSVFGVGLKTAKKWYEKGYRTLEEVKKDKNLKYTKMQKSGLEYYEDLNKPVSRAEAEAVEKIVKEAVKKYLPNAIVTSVGGFRRGKKIGHDVDILITTPEEENKLKELLKKVVEYLEEKGLLLYKDLVESTFEKFKLPSRQVDTLDHFDKCFMIIKLYDADVDPSLSQYNEKKDWRAVRVDLVIAPYDVYAFALLGWTGSRQFERDIRRYATHEKNMLLDNHSLYDITNRKFLEAKSEEEIFKHLGLEYVEPSERNA

SEQ ID NO: 21 - protein, 389 aa, synthetic construct
MGHQLVVRTDYSATPNPGFQKTPPLAVEPVSQYACQRRTTLDNKNKKFTDAFETLAEYAEYKENEVSKVTFERAASVLKSLPKEIKSLKDIEGIPCLGDKSKKLIEEILENGYSKEVEKIKKDERYQKLKLFTSVFGVGLKTANKWIEKGYRKLEDVINDKNLKLTKMQKEGLKYYEDLTKPVSRAEAEAVKKIVEEAVYKYLPNAKVTLCGGFRRGKKIGHDVDILITSPEDEKKLKELLEKVVKYLEEKGLLLYHDLVESTFEKFKLPSRQVDTLDHFAKCFMIIKLYYSEVDPSISDTIEGKQWRAVRVDLVIAPYDQYAFALLGWTGSRQFERDIRRYATHEKNMALDNHGLYDLTRRERLEAKSEEEIFKHLGLEYVEPTERNA

SEQ ID NO: 22 - protein, 389 aa, synthetic construct
MGHQLVVRTDYSATPNPGFQKTPPLAVEKISQYACQRKTTLDNRNKKFTDAFEVLAEYEEYKENEVSKVTFERAASVLKSLPYEIKSIKDIDGIPCLGDKNKKIIEEILENGYSKEVEKLKKDERYQALKLFTSVFGVGLKTANKWYEKGYRTLEDVINDKNLKLTKMQKIGIKYYEDLSKPVSRAEAEAVMKIVKEAVHKFLPNAKVTMVGGFRRGKKIGHDVDILITAPENEEKLKELLEKVVKYLEEQGLLLYKDLVESTFEKFKLPSRQVDTLDHFSKCFMIIKLDLEEVDPSISPSIEGKKWRAVRVDLVIAPYDEYAFALLGWTGSRQFERDIRRYATHEKNMLLDNHGLYDLTTRKRLEAKSEEEIFKHLGLEYVEPKERNA

SEQ ID NO: 23 - protein, 389 aa, synthetic construct
MGHQLVVRTDYSATPNPGFQKTPPLAVEKISQYACQRKTTLDNKNKKFTDAYEVLAEYAEYKENEVSKVTFERAASVLKSLPKEIKSIEDLKGIPCLGDKTKKLIEEILENGKSKEVEKIKKDERYQILKLFTSVFGVGLKTANKWYNKGYRTLEDVINDKNLKLTKMQKSGIKYYEDLNKPVSRAEAEAVTKIVKEAVYKFLPNAQVTLVGGFRRGKKIGHDVDILITTPSKEEELKELLEKVVKYLEERGLLLYKDLVESTFEKFKLPSRQVDTLDHFAKCFMIIKLPLEYVDPKVSKYIEGKKWRAVRVDLVIAPYDRFAFALLGWTGSRQFERDIRRYATHEKNMLLDNHSLYDLTSRKYLEAKSEEEIFKHLGLEYVEPEERNA

SEQ ID NO: 24 - protein, 389 aa, synthetic construct
MGHQLVVRTDYSATPNPGFQKTPPLAVKPISQYACQRRTTLENKNEKFTDAFEVLAEYAEYKENEVSKVTFERAASVLKSLPKEIKSIEDLKGIPCLGDKIKKEIEEILENGYSKEVEKIKKDERYQTYKLFTSVFGVGLKTAKKWYEKGYRTLEEVINDKNLKFTKMQKNGIKYYEDLKRDVTRAEAEAVLGIVREAVKRFLPNAEVTLVGGFRRGKKIGHDVDVLITTPEEESKLHELLPKVLAYLEEQGLLLYYDLVESTFEKFKLPSRQVDTLDHFMKCFTIIKLPVEKVDPSLSPTLEGKKWRAVRVDLVLAPWEYRAFALLGWTGSRQFERDIRRYATHERNMLLDNHLLYDRTERRFLEARSEEEIFRHLGLEYVEPAERNA

SEQ ID NO: 25 - protein, 389 aa, synthetic construct
MGHQLVVRTDYSATPNPGFQKTPPLAVKPISQYACQRRTTLDNKNREFTDAFEVLAEYAEYKENEVSKVTFERAASVLKSLPHRINSMEDIEGIPCLGDKIKKLIEEILENGTSKEVEKIKKDERYQNLKLFTSVFGVGLKTAKKWIEKGYRTLEEVINDKNLKFTKMQKAGIKYYEDLTREVTRAEAEAVLGIVREAVHQFLPNATVTLVGGFRRGKKIGHDVDVLITSPEEEGKLRSLLPKVVELLEERGLLLYYDLVESTFEKFKLPSRQVDTLDHFQKCFLIIKLPDFLVDPSKSGKREGKKWRAVRVDLVLAPYERRAFALLGWTGSRQFERDIRRYATHERNMLLDNHSLYDTTKRKFLPAESEEEIFKHLGLEYVEPQERNA

SEQ ID NO: 26 - protein, 389 aa, synthetic construct
MGHQLVVRTDYSATPNPGFQKTPPLAVKKISQYACQRKTTLNNYNRIFTDAFEILAEYAEFKENEVSNVTFKRAASVLKSLPYRITSMEDTEGIPCLGDKVKGLIEEIIENGTSKEVEKIKNDERYQTFKLFTSVFGVGLKTAEKWYERGYRTLEEVISDKTLKFTKMQKAGLLYYEDLTRCVTRAEAEAVLVLVREAVWSFLPDANVTMTGGFRRGKKIGHDVDFLITSPGEEGKLESLLPKVVTLLEERGLLLYYDLVESTFEKFKLPSRQVDTLDHFQKCFLIVKLEHQRVDSSKSEHREGKDWRAIRVDLVVAPYERRAFALLGWTGSRQFERDIRRYATHERNMILDNHRLYDRTKRQFLKAESEEEIFAHLGLDYVEPSERNA

SEQ ID NO: 27 - protein, 389 aa, synthetic construct
MGHQLVVRTDYSATPNPGFQKTPPLAVKPISQYACQRRTTLDNKNYKFTDAFEVLAEYAEYKENEVSKVTFERAASVLKSLPYEIKSIEDLKGIPCLGDKIKKLIEEILENGYSKEVEKIKKDERYQTYKLFTSVFGVGLKTAKKWYEKGYRTLEEVINDKNLKFTKMQKNGIKYYEDLKRDVSRAEAEAVLTIVREAVRRFLPNAEVTLVGGFRRGKKIGHDVDVLITSPEEESKLRELLPKVVAYLEEQGLLLYYDLVESTFEKFKLPSRQVDTLDHFRKCFMIIKLPVDWVDPSLSPFLEGKKWRAVRVDLVLVPHEARAFALLGWTGSRQFERDIRRYATHERDMLLDNHWLYDRTARRFLPAESEEEIFRHLGLPYVEPAERNA

SEQ ID NO: 28 - protein, 389 aa, synthetic construct
MGHQLVVRTDYSATPNPGFQKTPPLAVKPISQYACQRRTTLENKNKKFTDAFEVLAEYAEYKENEVSKVTFERAASVLKSLPYEIKSIEDCKGIPCLGDKILKLIEEILENGYSEEVKKIEKDERYQTYKLFTSVFGVGLKTAKKWYEKGIRTLEEYINNKNLKLTKMQKYGIKYYEDLNKPVTRAEAEAILEIVKEAVKKYLPDAEVTQVGGFRRGKKIGHDVDVLITSPSDESKLKELLEKVVKDLEEKGLLLYYDLVESTFEKFKLPSRQVDTLDHFAKCFMIIKLYLEKVDPKLSKNIEKKKWRAVRVDLVVAPYDYKAFALLGWTGSRQFERDIRRYATHEKNMLLDNHGLYDTTQRKFLEAKSEEEIFQHLGLEYVEPAERNA

SEQ ID NO: 29 - protein, 389 aa, synthetic construct
MGHQLVVRTDYSATPNPGFQKTPPLAVKPISQYACQRRTTLDNKNKKFTDAFEVLAEYYEYKENEVSKVTFKRAASVLKSLPKEIKSFEDVKGIPCLGDKNRKLIEEILENGYSEEVKKIEKDERYQAYKLFTSVFGVGLKTAKKWVEKGYRTLEEYINDKNLKLTKMQKCGIKYYEDLKAPVTRAEAEAILKIVKEAVKKYLPDAEVTLVGGFRRGKKIGHDVDVLITSPSDESKLKELLKKVVKDLEEKGLLLYYDLVESTFEKFKLPSRQVDTLDHFAKCFMIIKLPIDMVDPKLSEYIEEKKWRARRVDLVLAPYDRKAFALLGWTGSRQFERDIRRYATHEKNMLLDNHRLYDTTQRKFLEAKSEEEIFEHLGLEYVEPSERNA

SEQ ID NO: 30 - protein, 389 aa, synthetic construct
MGHQLVVRTDYSATPNPGFQKTPPLAVEKISQYACKRKTTLKNYNKKFTDAFEILAENAEYKENEVSYVTYKRAASVLKSLPFTIISMEDTEGIPCLGDKIKKIISEIIKDGYSSEVEKVLNNEEYKSFKLFTSVFGVGLKTAKKLFEKGYRTLEDIINDKSLKFTKMQKAGFLYYEDLVSPVTREEAEAVGVLVKEAVHAFLPDAFVEMVGGFRRGKKIGHDVDFLIYSKGSAEKEETLLQKVIDLWKKKGILLYYDLVESTFEKFKLPSRQVDTLDHFQKCFLILKLEHQRVDSSKSSHMEGKTWKAVRVDLVLAPFENYAFALLGWTGSRQFERDIRRYATHERKMMLDNHRLYDKEKREFLKADSVEEIFKHLGLEYIEPHERNA

SEQ ID NO: 31 - protein, 389 aa, synthetic construct
MGHQLVVRTDYSATPNPGFQKTPPLAVEKISQYACKRKTTLKNYNKKFTDAFEILAENAEYKENEVSYVTYKRAASVLKSLPFTIISMEDTEGIPCLGDKIKCIISEIINDGYSSEVEKVLNNEEYKSFKLFTSVFGVGLKTAKKWFEKGYRTLEDIINDKSLKFTKMQKAGFLYYEDLVSPVTREEAEAVGVLVKEAVHAFLPDAFVEMTGGFRRGKKIGHDVDFLISSAGSAEKEETLLQKVIDLWKKKGILLYYDLVESTFEKFKLPSRQVDTLDHFQKCFLILKLEHQRVDSSKSSHMEGKTWKAVRVDLVLAPWENYAFALLGWTGSRQFERDIRRYATHERKMMLDNHRLYDKEKREFLKAESVEEIFEHLGLEYIEPHERNA

SEQ ID NO: 32 - protein, 389 aa, synthetic construct
MGHQLVVRTDYSATPNPGFQKTPPLAVKKISQYACQRKITLNNYNHIFTDAFEILAEMAEFKENEVSYVTFMRAASVLKSLPFTITSMKDTEGIPCLGDKVKCIIEEIIEDGESSEVKAVLNDERYQSFKLFTSVFGVGLKTAEKWFRMGHRSLSDIMKDKTIKFTKMQKAGFLYYEDLRTCITRTEAEAIGVIVKEAVWAFDPDAFVIMTGGFRRGKKIGHDVDFVITSPGSWEDERQLLPKVIRWCEKKGHLLYYDLVESTFEKFKLPSRQVDTLDHFQKCFMILKLHFWWRDPSKSNQCEGKQWKACRVDLVMCHWEHRAFALLGWTGSRQFERDIRRYATHERKMMLDNHALYDKTKWVFLKAESEEEIFRHLGLPYIEPWERNA

SEQ ID NO: 33 - protein, 389 aa, synthetic construct
MGHQLVVRTDYSATPNPGFQKTPPLAVKKISQYACQRKITLNNYNHIFTDAFEILAEMAEFKENEVSYVTFMRAASVLKSLPFTITSMKDTEGIPCLGDKVKCIIEEIIEDGESSEVNKVLNDERYQSFKLFTSVFGVGLKTAEKWFRMGHRSLSDILKDKTIKFTKMQKAGFLYYEDLRSCITRTEAEAIGVIVKEAVWAFDPDAFVIMTGGFRRGKKIGHDVDFVITSPGSWECEEQLLPKVIRWCEKKGHLLYYDLVESTFEKFKLPSRQVDTLDHFQKCFMILKHHWWWRDPSKSNQCEGKQWKACRVDLVVCHWEHRAFALLGWTGSRQFERDIRRYATHERKMMLDNHALYDKTKWVFLKAESEEEIFEHLGLPYIEPWERNA

SEQ ID NO: 34 - protein, 389 aa, synthetic construct
MGHQLVVRTDYSATPNPGFQKTPPLAVKKISQYACQRKITLNNYNHIFTDAFEILAEMAEFKENEVSYVTFMRAASVLKSLPFTITSMKDTEGIPCLGDKVKCIIEEIIETGESSEVNAVLNDERYQSMKLFTSVFGVGLKTAEKWFRMGHRSLSDILKDKTIKFTKMQKAGFLYYEDLRSCVTRAEADAIEVIVKEAVWAFDPDAFVIMTGGFRRGKKIGHDVDFVITSPGSWECERQLLPKVIRWCEKKGHLLYYDLVESTFEKFKLPSRQVDTLDHFQKCFMILKLHMWWVDPSKSNQCEGKQWKAIRVDLVMCHWEHRAFALLGWTGSRQFERDIRRYATHERKMMLDNHALYDKTKWVFLKAESEEEIFEHLGLPYIEPWERNA

SEQ ID NO: 35 - protein, 389 aa, synthetic construct
MGHQLVVRTDYSATPNPGFQKTPPLAVKKISQYACQRKITLNNYNHIFTDAFEILAEMAEFKENEVSHVTFMRAASVLKSLPFTITSMKDTEGIPCLGDKVKCIIEEIIETGESSEVKKVLNDERYQSFKLFTSVFGVGLKTAEKWYRWGHRSLSDILKDKTIKFTKMQKAGFLYYEDLKQCITRAEAEAIGVIVKEAVWAFDPDAFVIMTGGFRRGKKIGHDVDFVITSPGSAECERRLLPKVIRWCEKKGHMLYYDLVESTFEKFKLPSRQVDTLDHFQKCFMILKLHMWWVDPSKSNQCEGKGWKACRVDLVVCHWEHRAFALLGWTGSRQFERDIRRYATHERGMMLDNHALYDKTKWVFLKAESEEEIFEHLGLPYIEPWERNA

SEQ ID NO: 36 - protein, 389 aa, synthetic construct
MGHQLVVRTDYSATPNPGFQKTPPLAVKKISQYACQRKITLNNYNHIFTDAFEILAEMAEFKENEVSHVTFMRAASVLKSLPFTITSMKDTEGIPCLGDKVKCIIREIIETGESSEVEAVLNDERYQAFKLFTSVFGVGLKTAEKWYRWGFRSLSDILKDKTLKFTKMQKAGFLYYEDLSSCVTRTEAEAIGKIVKEAVWAFDPDAFVIMTGGFRRGKKIGHDVDFVITSPGPSEMEEQLLPKVINWMEKKGHLLYYDLVESTFEKFKLPSRQVDTLDHFQKCFMILKLHYWWRDPSKSNQCEGKQWKAIRVDLVVCHWEHRAFALLGWTGSRQFERDIRRYATHERGMMLDNHGLYDRTKWVFLKAESEEEIFEHLGLPYIEPWERNA

SEQ ID NO: 37 - protein, 389 aa, synthetic construct
MGHQLVVRTDYSATPNPGFQKTPPLAVKKISQYACQRKITLNNYNHIFTDAFEILAEMAEFKENEVSHVTFMRAASVLKSLPFTITSMKDTEGIPCLGDKVKCIIREIIETGTSSEVEAVLNDERYQAFKLFTSVFGVGLKTAEKWYRMGHRSLSDIRKDKSIKFTKMQKAGFIYYEDLSSCITRAEADAIEKIVKEACWAFDPDAKVIMTGGFRRGKKIGHDVDFVITSPGPSEMERQLLPKMINWCEKQGYLLYYDLVESTFEKFKLPSRQVDTLDHFQKCFMILKLHMKRVDSSKSNQCEGKGWKACRVDLVMCHWEHRAFALLGWTGSRQFERDIRRYATHERGMMLDNHGLYDRTKWTFLKAESEEEIFRHLGLPYIEPWERNA

SEQ ID NO: 38 - protein, 389 aa, synthetic construct
MGHQLVVRTDYSATPNPGFQKTPPLAVKKISQYACQRKITLNNYNHIFTDAFEILAEMAEFKENEVSYVTFMRAASVLKSLPFTITSMKDTEGIPCLGDKVKCIIREIIETGHSSEVEAVLNDERYQAFKLFTSVFGVGLKTAEKWYRWGHRSLSDIRKDKSIKFTKMQKAGFKYYEDLSSRVTRAEAEAIAKIVKEATWAFDPDAFVIMTGGFRRGKKIGHDVDFVITSPGPSEMERRLLPWIINWMWKQGHMLYYDLVESTFEKFKLPSRQVDTLDHFQKCFMILKLHMKRVDSSKSNQCEGKNWKAIRVDLVVCHWEHRAFALLGWTGSRQFERDIRRYATHERGMMLDNHGLYDRTKHTFLKAESEEEIFEHLGLEYIEPWERNA

SEQ ID NO: 39 - protein, 389 aa, synthetic construct
MGHQLVVRTDYSATPNPGFQKTPPLAVKKISQYACQRKITLNNYNHIFTDHFEILAEMAEFKENEVSHVTFMRAAAVLKSLPFTITSMKDTEGIPCLGDKVKRIIREIIETGTSSEVENVLNDERYQAFKLFTSVFGVGLKTAEKWYRWGHRSLCDIRKDKSIKFTKMQKAGFKYYEDLSSRITRDEAEAIAKIVKEATWAFDPDAEVQMTGGFRRGKKIGHDVDFVITSPGPEWMEWQLLPWIINWMMKQGHMLYYDLVESTFEKFKLPSRQVDTLDHFQKCFMILKLHMKHVDPSQSNQNEGRHWKACRVDLVVCHWEHRAFALLGWTGSRQFERDIRRYATHERGMMLDNHGLYDRTRHTFLKAETEKEIFEHLGLEYIEPWERNA

SEQ ID NO: 40 - protein, 389 aa, synthetic construct
MGHQLVVRTDYSATPNPGFQKTPPLAVKKISQYACQRKITLCNHNKIFTDAFEILAEMAEFKENEVSYVTYMRAAAVLKSLPFTITSMKHTEGIPCLGDKVKRIIKEIIETGHSSEVENVLNDERYQAFKLFTSVFGVGLKTAEKWYRMGHRSLEDIRKDKSIKLTKMQKAGFKYYDDLSSRITRDEAEAIAKIVKEATWAFDPDAVVVMCGGFRRGKKIGHDVDFVITSPGPDSMEMNLLPWMINYWMKQGYMLYYDLVESTFEKFKLPSRQVDTLDHFQKCFCILMLHFKYRDSSQSDCQEGQNWKACRVDLVMCHWEHRAFALLGWTGSRQFERDIRRYATHERGMMLDNHGLYDRTRHTFLKAESEKEIFEHLGLEYIEPRERNA

SEQ ID NO: 41 - protein, 389 aa, synthetic construct
MGHQLVVRTDYSATPNPGFQKTPPLAVKKISQYACQRKTTLNNCNHIFTDAFEILAENYEFRENEVSYLTFMRAASVLKSLPFTIISMKDTEGIPCLGDKVKCIIEEIIEDGESSEVKAVLNDERYQSFKLFTSVFGVGLKTSEKWFRMGFRSLSKIRSDKTLKFTRMQKAGFLYYEDLVSCVTRAEAEAVGVLVKEAVWAFLPDAFVTMTGGFRRGKKIGHDVDFLITSPGSTEDEEQLLPKVINLWEKKGLLLYYDLVESTFEKFKLPSRQVDTLDHFQKCFLILKLHHQRVDSGKSNQQEGKTWKAIRVDLVMCPYENRAFALLGWTGSRQFERDIRRYATHERKMMLDNHALYDKTKRIFLKAESEEEIFAHLGLDYIEPWERNA

SEQ ID NO: 42 - protein, 389 aa, synthetic construct
MRHQLVVRTDYSASPNPGFQKTPPLAVKKISQYACQRKTTLNNCNRIFTDAFEVLAENYEFRENEVFCLAFMRAASVLKSLPFTIISMKDTEGIPCLGDKVKCIIEEIIEDGESSEVKAVLNDERYKSFKLFTSVFGVGLKTSEKWFRMGFRTLSKIRSDKTLKFTRMQKAGFLYYEDLVSCVTRAEAEAVSVLVKEAVWAFLPDAFVTMTGGFRRGKKTGHDVDFLITSPGSTEDEEQLLPKVINLWERKGLLLYYDLVESTFEKLKLPSRKVDALDHFQKCFLILKLHHQRVDSGKSNQQEGKTWKAIRVDLVMCPYENRAFALLGWTGSRQFERDLRRYATHERKMILDNHALYDKTKRIFLKAESEEEIFAHLGLDYIEPWERNA

SEQ ID NO: 43 - protein, 389 aa, synthetic construct
MHHLLVVRTDYSATPNPGFQKTPPLAVKKISQYACQRKTTLNNCNHIFTDAFEVLAENYEFRENEVFCLAFMRAASVLKSLPFTIISMKDTEGIPCLGDKVKCIIEEIIEDGESSEVKAVLNDERYKSFKLFTSVFGVGLKTSEKWFRMGFRTLSKIRSDKTLKFTRMQKAGFLYYEDLVSCVTRAEAEAVSVLVKEAVWAFLPDAFVTMTGGFRRGKKTGHDVDFLITSPGSTEDEEQLLPKVINLWERKGLLLYYDLVESTFEKLKLPSRKVDALDHFQKCFLILKLHHQRVDSGKSNQQEGKTWKAIRVDLVMCPYENRAFALLGWTGSRQFERDLRRYATHERKMILDNHALYDKTKRIFLKAESEEEIFAHLGLDYIEPWERNA

SEQ ID NO: 44 - protein, 389 aa, synthetic construct
MHHLLVVRTDYSATPNPGFQKTPPLAVKKISQYACQRKTTLNNCNHIFTDAFEILAENYEFRENEGSYVAFMRAASVLKSLPFTIISMKDTEGIPCLGDKVKCIIEEIIEDGESSEVKAVLNDERYQSFKLFTSVFGVGLKTSEKWFRMGFRTLSKIRSDKTLKFTRMQKAGFLYYEDLVSCVTRAEAEAVGVLVKEAVRAFLPDAFVTMTGGFRRGKKIGHDVDFLITSPGSAEDEEQLLPKVINLWERKGLLLYCDLVESTFEKLKLPSRKVDALDHFQKCFLILKLHHQRVDSGKSNQQEGKTWKAIRVDLVMCPYENRAFALLGWTGSRQFERDLRRYATHERKMMLDNHALYDKTKRIFLKAESEEEIFAHLGLDYIEPWERNA

SEQ ID NO: 45 - protein, 389 aa, synthetic construct
MHHLLVVRTDYSASPNPGFQKTPPLAVKKISPYACQRKTTLNNCNHIFTDAFEVLAENYEFRENEGFYLAFMRAASVLKSLPFTIISMKDTEGIPCLGDKVKCIIEEIIEDGESSEVKAVLNDERYQSFKLFTSVFGVGLKTSEKWFRMGFRSLSKIRSDKTLKFTRMQKAGFLYYEDLVSCVTRAEAEAVSVLVKEAVRAFLPDAFVTMTGGFRRGKKIGHDVDFLITSPGSAEDEEQLLPKVINLWERKGLLLYSDLVESTFEKLKLPSRKVDALDHFQKCFLILKLHHQRVDSGKSNQQEGKTWKAIRVDLVMCPYENRAFALLGWTGSRQFERDIRRYATHERKMMLDNHALYDKTKRIFLKAESEEEIFAHLGLDYIEPWERNA

SEQ ID NO: 46 - protein, 389 aa, synthetic construct
MHHQLVVRTDYSASPNPGFQKTPPLAVKKISQYACQRKTTLNNCNHIFTDAFDILAENYEFKENEVSYLAFMRAASVLKSLPFTIISMKDTEGIPCLGDKVKCIIEEIIEDGESSEVKAVLNDERYQSFKLFTSVFGVGLKTSEKWFRMGFRTLSKIRSDKTLKFTRMQKAGFLYYEDLVSCVTRAEAEAVGVLVKEAVWAFLPDAFVTMTGGFRRGKKIGHDVDFLITSPGSTEDEEQLLPKVINLWERKGLLLYCDLVESTFEKFKLPSRKVDALDHFQKCFLILKLHHQRVDSGKSNQQEGKTWKAIRVDLVMCPYENRAFALLGWTGSRQFERDLRRYATHERKMMLDNHALYDKTKRIFLKAESEEEIFAHLGLDYIEPWERNA

SEQ ID NO: 47 - protein, 389 aa, synthetic construct
MRHQLVVRTDYSATPNPGFQKTPPLAVKKISQYACQRKTTLNNCNHIFTDAFEVLAENYEFRENEVFYLTFMRAASVLKSLPFTIISMKDTEGIPCLGDKVKCIIEEIIEDGESSEVKAVLNDERYKSFKLFTSVFGVGLKTSEKWFRMGFRSLSKIRSDKTLKFTRMQKAGFLYYEDLVSCVTRAEAEAVGVLVKEAVWAFLPDAFVTMTGGFRRGKKTGHDVDFLITSPGSAEDEEQLLPKVINLWERKGLLLYCDLVESTFEKLKLPSRKVDALDHFQKCFLILKLHHQRVDSGKSNQQEGKTWKAIRVDLVMCPYENRAFALLGWTGSRQFERDLRRYATHERKMMLDNHALYDKTKRIFLKAESEEEIFAHLGLDYIEPWERNA

SEQ ID NO: 48 - protein, 389 aa, synthetic construct
MGHQLVVRTDYSATPNPGFQKTPPLAVKKISQYACQRRTTLNNYNHIFTDAFEILAENSEFRENEVSYVTFMRAASVLKSLPFTIISMKDTEGIPCLGDKVKCIIEEIIEDGESSEVKAVLNDERYQSFKLFTSVFGVGLKTSEKWFRMGFRSLSKIRSDKTLKFTKMQKAGFLYYEDLVSCVTRAEAEAVGVLVKEAVWAFLPDAFVTMTGGFRRGKKIGHDVDFLITSPGSAEDEEQLLPKVINLWEKKGLLLYYDLVESTFEKFKLPSRQVDTLDHFQKCFLILKLHHQRVDSSKSNQQEGKTWKAIRVDLVMCPYERRAFALLGWTGSRQFERDIRRYATHERKMMLDNHALYDKTKRVFLKAESEEEIFAHLGLDYIEPWERNA

SEQ ID NO: 49 - protein, 389 aa, synthetic construct
MGHQLVVRTDYSATPNPGFQKTPPLAVKKISQYACQRKTTLNNCNHIFTDAFEILAENYEFRENEVSYVTFMRAASVLKSLPFTIISMKDTEGIPCLGDKVKCIIEEIIEDGESSEVKAVLNDERYQSFKLFTSVFGVGLKTSEKWFRMGFRSLSKIRSDKTLKFTRMQKAGFLYYEDLVSCVTRAEAEAVGVLVKEAVWAFLPDAFVTMTGGFRRGKKIGHDVDFLITSPGSAEDEEQLLPKVINLWEKKGLLLYYDLVESTFEKFKLPSRKVDALDHFQKCFLILKLHHQRVDSGKSNQQEGKTWKAIRVDLVMCPYENRAFALLGWTGSRQFERDIRRYATHERKMMLDNHALYDKTKRIFLKAESEEEIFAHLGLDYIEPWERNA

SEQ ID NO: 50 - DNA, 14 bp, synthetic construct
  source 1..14: mol_type = other DNA
aatacaacctctca

SEQ ID NO: 51 - DNA, 1167 bp, Bos taurus
  source 1..1167: mol_type = genomic DNA
atgaagcatcagctggttgttcgtaccgattatagcgcaaccccgaatccgggttttcagaaaacaccgcctctggcagttaaaaagattagccagtatgcatgtcagcgtaaaaccacgctgaataactataaccacattttcaccgatgcctttgaaattctggcagaaaacagcgaattcaaagaaaacgaagttagctacgtgacctttatgcgtgcagcaagcgttctgaaaagcctgccgtttaccattattagcatgaaagataccgaaggtattccgtgtctgggtgataaagtgaaatgcatcattgaagagatcatcgaagatggtgaaagcagcgaagttaaagcagttctgaatgatgaacgttaccagagcttcaaactgtttaccagcgtttttggtgttggcctgaaaaccagcgaaaaatggtttcgtatgggttttcgtagcctgagcaaaatcatgagcgataaaaccctgaaattcaccaaaatgcagaaagccggtttcctgtattatgaagatctggttagctgtgttacccgtgccgaagccgaagcagttggtgttctggttaaagaagcagtttgggcatttctgccggatgcatttgttaccatgaccggtggttttcgtcgtggtaagaaaattggtcatgatgtggattttctgattaccagtccgggtagcgcagaagatgaagaacagctgctgccgaaagttattaatctgtgggaaaagaaaggtctgctgctgtattacgatctggttgaaagcaccttcgagaaattcaaactgccgagccgtcaggttgataccctggatcactttcagaaatgttttcttatcctgaagctgcatcatcagcgtgttgatagcagcaaaagcaatcagcaagaaggtaaaacctggaaagcaattcgtgttgatctggtgatgtgtccgtatgaaaatcgtgcatttgcactgttaggttggaccggtagtcgtcagtttgaacgtgatattcgtcgttatgcaacccatgaacgtaaaatgatgctggataatcatgccctgtacgataaaacgaaacgcgtgttcctgaaagccgaaagcgaagaagaaatttttgcacatctgggccttgattacattgaaccgtgggaacgtaatgca

SEQ ID NO: 52 - DNA, 1167 bp, synthetic construct
  source 1..1167: mol_type = other DNA
atgggtcatcagctggttgttcgtaccgattatagcgcaaccccgaatccgggttttcagaaaacaccgcctctggcagttaaaaagattagccagtatgcatgtcagcgtaaaaccacgctggataacaaaaacaaaaagtttaccgatgcgctggaagaactggcagaatatgaagaatataaagaaaacgaggtgagcaaggtgacctttgaacgtgcagcaagcgttctgaaaagcctgccgtttgaaatcaaaagcctgaaagatctggaaggtattccgtgtctgggtgacaaaattaagaaactgattgaagaaatcctggaaaacggctatagcaaagaagtggaaaagatcaaaaaggacgaacgttatcagaccctgaaactgtttaccagcgtttttggtgttggcctgaaaaccgcaaagaaatggtatcgtaaaggttatcgtaccctggaagaagtgaaaaacgataagaccttaaagctgaccaaaatgcagaaagcaggcctgaaatattacgaagatctgaccagcggtgttacccgtgcagaagcagaagcaattctggttattgttaaagaagcagttcacgcatttctgccggatgccgaagttaccctggttggtggttttcgtcgtggtaagaaaattggtcatgatgtggatgttctgattaccagtccgggtcctgcagaggatctggaacagctgctgccgaaagttgttaattatctggaagaaaaaggcctgctgctgtattatgatctggttgaaagcaccttcgagaaattcaaactgccgagccgtcaggttgataccctggatcattttgccaaatgcttcatgatcattaaactgccgcatcagtgggttgatccgagcctgagcaatcagcaagaaggtaaaacctggaaagcagttcgtgttgatctggtgctggcaccgtatgaaaatcgtgcatttgcactgttaggttggaccggtagtcgtcagtttgaacgcgatattcgtcgttatgcaacccatgagaaaaatatgctgctggataatcatggcctgtacgataaaaccaaacgcgtgtttctgaaagccgaaagcgaagaagaaatttttgcacatctgggccttgattatgttgaaccgtgggaacgtaatgca

SEQ ID NO: 53 - DNA, 1167 bp, synthetic construct
  source 1..1167: mol_type = other DNA
atgggtcatcagctggttgttcgtaccgattatagcgcaaccccgaatccgggttttcagaaaacaccgcctctggcagttgagaaaatttcacagtatgcatgtcagcgtaaaaccacgctgaaaaacctgaacaaaaagtttaccgatgcctttgaaatcctggcagaatatgccgaatataaagaaaacgaagtgagcaaagtgacctttgaacgtgcagcaagcgttctgaaaagcctgccgtttgagattaaaagcatggaagataccgaaggtattccgtgtctgggtgataaaattcgcaaaatcattgaagagatcctggaaaaaggttatagcagcgaagttgaaaaagtgctgaaagatgaacgttaccaggcctttaaactgtttaccagcgtttttggtgttggcctgaaaaccgcaaagaaatggtatgaaaaaggctatcgtacccttgaggatatcaaaaaggataagagcctgaagttcaccaaaatgcagaaagcaggcttcaaatattacgaagatctggttgcaccggttacacgtgcagaagcagaagccgttggtaaactggttgaagaagcagttcacgaatttctgccggatgcaaaagttaccatggttggtggttttcgtcgtggtaaaaagattggtcatgatgtggattttctgattaccacaccgggtgaagaagagaaagttaaagaactgctgaaaaaggtgattgacctgtgggaaaagaaaggtctgctgctgtattatgatctggtggaaagcaccttcgagaaattcaaactgccgagccgtcaggttgataccctggatcattttgaaaaatgctttatgatcctgaaactgcattacaaagaagtggatccgagcgttagcagccatatggaaggtaagaaatggaaagcagttcgtgttgatctggtagcagcaccgtatgaaaattatgcatttgcactgttaggttggaccggtagtcgtcagtttgaacgcgatattcgtcgttatgcaacccatgaacgtaatatgctgctggataatcatcgtctgtatgatctgaccaaacgtgaattcctggaagccaaaagcgaagaagaaatctttgaacatctgggccttgagtatattgaaccgcatgaacgcaatgca

SEQ ID NO: 54 - DNA, 1167 bp, synthetic construct
  source 1..1167: mol_type = other DNA
atgggtcatcagctggttgttcgtaccgattatagcgcaaccccgaatccgggttttcagaaaacaccgcctctggcagttgagaaaatttcacagtatgcatgtcagcgtaaaaccacgctgaaaaacctgaacaaagaatttaccgatgcctttgaaatcctggcagaatatgccgaatataaagaaaacgaagtgagcaaagtgacctttgaacgtgcagcaagcgttctgaaaagcctgccgtttaaaatcgaaagcatggaagataccgaaggtattccgtgtctgggtgataaaattcgcaaaatcattgaagagatcctggaaaaaggctatagcgaagaagttcgtaaagtcctggaagatgaacgttatcaggcctttaaactgtttaccagcgtttttggtgttggcctgaaaaccgcaaagaaatggtatgaaaaaggttatcgtacccttgaggacatcaaaaaggataaaagcctgaagttcaccaagatgcagaaagcaggctttaaatactatgaagatctggttgcaccggttacacgtgcagaagcagaagccgttggtaaactggttgaagaagcagttcacgaatttctgccggatgcaaaagttaccatggttggtggttttcgtcgtggtaaaaagattggtcatgatgtggattttctgattaccacaccgggtgaagaagagaaagttaaagaactgctgaagaaagtgattgagctgtgggaaaagaaaggtctgctgctgtattatgatctggtggaaagcaccttcgagaaattcaaactgccgagccgtcaggttgataccctggatcattttgaaaaatgctttatgatcctgaagctgccgtatgaactggtagatccgagcgttagcagccatatggaaggtaagaaatggaaagcagttcgtgttgatctggtagcagcaccgtatgaaaattatgcatttgcactgttaggttggaccggtagtcgtcagtttgaacgcgatattcgtcgttatgcaacccatgaacgtaatatgctgctggataatcatcgtctgtatgatctgaccaaacgcgaattcctgaaagccgaatcagaagaggaaatctttaaacatctgggccttgagtatatcgaaccgcatgaacgcaatgca

SEQ ID NO: 55 - DNA, 1167 bp, synthetic construct
  source 1..1167: mol_type = other DNA
atgggtcatcagctggttgttcgtaccgattatagcgcaaccccgaatccgggttttcagaaaacaccgcctctggcagttgagaaaatttcacagtatgcatgtcagcgtaaaaccacgctgaaaaacctgaacaaagaatttaccgatgcctttgaaatcctggcagaatatgccgaatataaagaaaacgaagtgagcaaagtgacctttgaacgtgcagcaagcgttctgaaaagcctgccgtttaaaatcgaaagcatggaagataccgaaggtattccgtgtctgggtgataaaattcgcaaaatcattgaagagatcctggaaaaaggctatagcgaagaagttgagaaggtcctgaaagatgaacgttatcaggcctttaaactgtttaccagcgtttttggtgttggcctgaaaaccgcaaagaaatggtatgaaaaaggttatcgtaccctggaagatatcaaaaaggacaaaagcctgaagttcaccaaaatgcagaaagccggtttcaaatattacgaagatctggttgcaccggttacacgtgccgaagccgaagcagttggtgttctggttaaagaagcagtgcataaatttctgccggatgcaaaagttaccatggttggtggttttcgtcgtggtaaaaagattggtcatgatgtggattttctgattaccacaccgggtgaagaagagaaagttaaagaactgctgaagaaagtgatcgacctgtgggaaaaagaaggtctgctgctgtattatgatctggtggaaagcaccttcgagaaattcaaactgccgagccgtcaggttgataccctggatcattttgaaaaatgctttctgatcctgaaactggactataaacgtgttgatccgagcgttagcagccatatggaaggtaagaaatggaaagccgttcgtgttgacctggttgcagcaccgtatgaaaattatgcatttgcactgttaggttggaccggtagtcgtcagtttgaacgcgatattcgtcgttatgcaacccatgaacgtaatatgctgctggataatcatcgtctgtatgatctgaccgaacgcaaatttctggaagccaaatcagaagaagaaatctttgaacatctgggccttgagtatattgaaccgcatgaacgcaatgca

SEQ ID NO: 56 - DNA, 1167 bp, synthetic construct
  source 1..1167: mol_type = other DNA
atgggtcatcagctggttgttcgtaccgattatagcgcaaccccgaatccgggttttcagaaaacaccgcctctggcagttgagaaaatttcacagtatgcatgtcagcgtaaaaccacgctgaataacctgaacaaagaatttaccgatgcctttgaaattctggcagaagatgccgaatataaagaaaacgaagttagcaaagtgacctttgaacgtgcagcaagcgttctgaaaagcctgccgtttaaaatcgaaagcatggaagataccgaaggtattccgtgtctgggtgataaaattcgctatatcattgaagaaatcctggaaaaaggctatagcagcgaagttctggaagtgctgaatgatgaacgttatcaggcctttaaactgtttaccagcgtttttggtgttggcctgaaaaccgcaaagaaatggtatgaaaaaggttatcgtaccctggaagatatcaaaaaggacaaaagcctgaagttcaccaaaatgcagaaagccggtttcaaatattacgaagatctggttgcagatgttacccgtgccgaagccgaagcagttggtgttctggttaaagaagcagtgcataaatttctgccggatgcactggttaccatggttggtggttttcgtcgtggtaaaaagattggtcatgatgtggattttctgattaccacaccgggtgatcaagaaaaactgaaagaactgctgaagaaagtgatcgatctgtgggaaaaagaaggtctgctgctgtattatgatctggtggaaagcaccttcgagaaattcaaactgccgagccgtcaggttgataccctggatcattttgaaaaatgctttctgatcctgaaactgcatcatgttcgtgttgatccgagcaaaagtctgtttatggaaggcaagaaatggaaagcagttcgtgtggatctggtagcagcaccgtatgaaaattatgcatttgcactgttaggttggaccggtagtcgtcagtttgaacgcgatattcgtcgttatgcaacccatgaacgtaatatgcagctggataatcatcgtctgtatgatgaaaccaaacgcgaattcctggaagccaaaagcgaagaagaaatctttgaacatctgggccttgagtatattgaaccgcatgaacgcaatgca

SEQ ID NO: 57 - DNA, 1167 bp, synthetic construct
  source 1..1167: mol_type = other DNA
atgggtcatcagctggttgttcgtaccgattatagcgcaaccccgaatccgggttttcagaaaacaccgcctctggcagttaaaaagattagccagtatgcatgtcagcgtaaaaccacactgaaaaacctgaacaaagaattcaccgatgcctttgaaattctggcagaatatgccgagtataaagaaaacgaagttagcaaagtgacctttgaacgtgcagcaagcgttctgaaaagcctgccgtttaaaatcgaaagcatggaagataccgaaggtattccgtgtctgggtgataaaatcaaaaagatcatcgaagaaatcctggaaaaaggctatagcgaagaggttaaaaaggtgctggaagatgaacgttatcaggcctttaaactgtttaccagcgtttttggtgttggcctgaaaaccgcaaagaaatggtatgaaaaaggttatcgtaccctggaagatatcaaaaaggacaaaagcctgaagttcaccaaaatgcagaaagccggtttcaaatattacgaagatctggttgcaccggttacacgtgccgaagccgaagcagttggtgttctggttcgtgaagcagttcatgcatttctgccggatgcatttgttaccatggttggtggttttcgtcgtggtaagaaaattggtcatgatgtggattttctgattaccacaccgggtagcgaagaagatcgtaaaaccctgctgccgaaagttattaatctgtgggaaaaacagggtctgctgctgtattatgatctggtggaaagcaccttcgagaaattcaaactgccgagccgtcaggttgataccctggatcattttgaaaaatgcttttgcatcctgaagctgcattatcagcgtgttgatccgagcgttagcaattttcaagaaggtaaaacctggaaagccgttcgtgtggatctggttctggcaccgtatgaaaattatgcatttgcactgttaggttggaccggtagtcgtcagtttgaacgcgatattcgtcgttatgcaacccatgaacgtaatatgctgctggataatcatcgtctgtatgatctgaccaaacgcgaatttctgaaagccgaaagtgaagaagaaatctttgcacatctgggccttgattacattgaaccgtgggaacgtaatgca

SEQ ID NO: 58 - DNA, 1167 bp, synthetic construct
  source 1..1167: mol_type = other DNA
atgggtcatcagctggttgttcgtaccgattatagcgcaaccccgaatccgggttttcagaaaacaccgcctctggcagttaaaaagattagccagtatgcatgtcagcgtaaaaccacgctggataacaaaaacaaaaagtttaccgatgcgctggaagaactggcagaatatgaagaatataaagaaaacgaggtgagcaaggtgacctttgaacgtgcagcaagcgttctgaaaagcctgccgtttgaaatcaaaagcatcaaagatctggaaggtattccgtgtctgggtgacaaaattaagaaactgattgaagaaatcctggaaaacggctatagcaaagaagtggaaaagatcaaaaaggacgaacgttatcagaccctgaaactgtttaccagcgtttttggtgttggcctgaaaaccgcaaagaaatggtatcgtaaaggttatcgtaccctggaagaagtgaagaaagataagaccttaaagctgaccaaaatgcagaaagcaggcctgaaatattacgaagatctgaccagcggtgttacccgtgcagaagcagaagcaattctggttattgttaaagaagcagttcacgcatttctgccggatgccgaagttaccctggttggtggttttcgtcgtggtaagaaaattggtcatgatgtggatgttctgattaccagtccgggtcctgcagaggatctggaacagctgctgccgaaagttgttaattatctggaagaaaaaggcctgctgctgtattatgatctggttgaaagcaccttcgagaaattcaaactgccgagccgtcaggttgataccctggatcattttgccaaatgcttcatgatcattaaactgccgcatcagtgggttgatccgagcctgagtccgcagattgaaggtaaaacatggaaagcagttcgtgttgatctggtgctggcaccgtatgaaaatcgtgcatttgcactgttaggttggaccggtagtcgtcagtttgaacgcgatattcgtcgttatgcaacccatgagaaaaatatgctgctggataatcaccgcctgtacgataaaaccaaacgcgtgtttctgaaagccgaaagcgaagaagaaatttttgcacatctgggccttgattatgttgaaccgtgggaacgtaatgca

SEQ ID NO: 59 - DNA, 1167 bp, synthetic construct
  source 1..1167: mol_type = other DNA
atgggtcatcagctggttgttcgtaccgattatagcgcaaccccgaatccgggttttcagaaaacaccgcctctggcagttaaaaagattagccagtatgcatgtcagcgtaaaaccacgctgaataacaagaacaaaaagtttaccgatgcgctggaaattctggccgaatatgaagaatataaagaaaacgaggtgagcaaggtgacctttgaacgtgcagcaagcgttctgaaaagcctgccgtttgaaatcaaaagcatcaaagatctggaaggtattccgtgtctgggtgacaaaattaagaaactgattgaagaaatcctggaaaacggctatagcaaagaagtggaaaagatcaaaaaggacgaacgttatcagaccctgaaactgtttaccagcgtttttggtgttggcctgaaaaccgcaaagaaatggtatcgtaaaggttatcgtaccctggaagaagtgatgaaagataaaaccctgaagttcaccaaaatgcagaaagccggtttcaaatattacgaggatctgaccagtccggttacacgtgccgaagccgaagcaattggtgttattgttaaagaagcagttcacgcatttctgccggatgccgaagttaccattgttggtggttttcgtcgtggtaagaaaattggtcatgatgtggatattctgattaccagtcctggtcctgcagaggatctggaacagctgctgccgaaagttgttaattatctggaagaaaaaggcctgctgctgtattatgatctggttgaaagcaccttcgagaaattcaaactgccgagccgtcaggttgataccctggatcattttgccaaatgcttcatgatcattaaactgccgcatcagtgggttgatccgagcctgagcaatcagcaagaaggtaaaacctggaaagcagttcgtgttgatctggtgctggcaccgtatgaaaatcgtgcatttgcactgttaggttggaccggtagtcgtcagtttgaacgcgatattcgtcgttatgcaacccatgagaaaaatatgctgctggataatcatggcctgtacgataaaaccaaacgcgtgtttctgaaagccgaaagcgaagaagaaatttttgcacatctgggccttgattatgttgaaccgtgggaacgtaatgca

SEQ ID NO: 60 - DNA, 1167 bp, synthetic construct
  source 1..1167: mol_type = other DNA
atgggtcatcagctggttgttcgtaccgattatagcgcaaccccgaatccgggttttcagaaaacaccgcctctggcagttaaaaagattagccagtatgcatgtcagcgtaaaaccacgctgaataactacaacaaaatcttcaccgatgcctttgaaattctggcagaaaacgccgaatttaaagaaaacgaagttagctacgtgacctttatgcgtgcagcaagcgttctgaaaagcctgccgtttaccattaaaagcatgaaagataccgaaggtattccgtgtctgggtgataaagtgaaaaagatcatcgaagaaatcatcgaggatggtgaaagcagcgaagttaaagcagttctgaatgatgaacgttaccagagcttcaaactgtttaccagcgtttttggtgttggcctgaaaaccagcgaaaaatggtttcgtatgggttttcgtagcctgagcgaaatcaaaagcgataaaaccctgaaattcaccaagatgcagaaagcgggttttctgtattatgaagatctggttagctgtgttacccgtgccgaagccgaagcagttggtgttctggttaaagaagcagttcacgcatttctgccggatgcatttgttaccattaccggtggttttcgtcgtggtaagaaaattggtcatgatgtggattttctgattaccagtccgggtagtccggaagatgaagaacagctgctgccgaaagttattaatctgtgggaaaagaaaggtctgctgctgtatagcgatctggttgaaagcacctttgagaaattcaaactgccgagccgtcaggttgataccctggatcactttcagaaatgttttcttatcctgaagctgcatcatcagcgtgttgatagcagcaaaagcaatcagcaagaaggtaaaacctggaaagcaattcgtgttgatctggttctgtgtccgtatgaacgtcgtgcatttgcactgttaggttggaccggtagtcgtcagtttgaacgtgatattcgtcgttatgcaacccatgaacgtaaaatgctgctggataatcatgccctgtatgataaaaccaaacgcgtgttcctgaaagccgaaagcgaagaagaaatttttgcacatctgggccttgattacattgaaccgtgggaacgtaatgca

SEQ ID NO: 61 - DNA, 1167 bp, synthetic construct
  source 1..1167: mol_type = other DNA
atgggtcatcagctggttgttcgtaccgattatagcgcaaccccgaatccgggttttcagaaaacaccgcctctggcagttaaaaagattagccagtatgcatgtcagcgtaaaaccacactgaataacctgaaccatatctttaccgatgcctttgaaattctggcagaaaacgccgaatataaagaaaacgaagttagctacgtgacctttatgcgtgcagcaagcgttctgaaaagcctgccgtttaaaatcatcagcatgaaagataccgaaggtattccgtgtctgggcgataaaatcaaatgcatcattgaagagattcttgaggatggtgaaagcagcgaagttaaagcagttctgaatgatgaacgttaccagagcttcaaactgtttaccagcgtttttggtgttggcctgaaaaccgcagaaaaatggtatcgtatgggttatcgtagcctgagcaaaatcatgagcgataaaaccctgaaattcaccaaaatgcagaaagccggtttcaaatattacgaagatctggttgcaccggttacacgtgccgaagccgaagcagttggtgttctggttaaagaagcagttcacgcatttctgccggatgcgtttgttaccatggttggtggttttcgtcgtggtaagaaaattggtcatgatgtggattttctgattaccagtccgggtagcgcagaagatgaagaacagctgctgccgaaagttattaatctgtgggaaaagaaaggtctgctgctgtattatgatctggtggaaagcaccttcgagaaattcaaactgccgagccgtcaggttgataccctggatcactttcagaaatgttttcttatcctgaagctgcatcatcagcgtgttgatagcagcaaaagcaatcagcaagaaggtaaaacctggaaagccgttcgtgttgatctggttatgtgtccgtatgaaaatcgtgcatttgcactgttaggttggaccggtagtcgtcagtttgaacgtgatattcgtcgttatgcaacccatgaacgtaatatgctgctggataatcatgccctgtatgataaaaccaaacgcgtgttcctgaaagccgaaagcgaagaagaaatttttgcacatctgggccttgattacattgaaccgtgggaacgtaatgca

SEQ ID NO: 62 - DNA, 1167 bp, synthetic construct
  source 1..1167: mol_type = other DNA
atgggtcatcagctggttgttcgtaccgattatagcgcaaccccgaatccgggttttcagaaaacaccgcctctggcagttaaaaagattagccagtatgcatgtcagcgtaaaaccacgctgaataactataaccacattttcaccgatgcctttgaaattctggcagaaaacgccgaatttaaagaaaacgaagttagctacgtgacctttatgcgtgcagcaagcgttctgaaaagcctgccgtttaccattattagcatgaaagataccgaaggtattccgtgtctgggtgataaagtgaaatgcatcattgaagagatcatcgaagatggtgaaagcagcgaagttaaagcagttctgaatgatgaacgttaccagagcttcaaactgtttaccagcgtttttggtgttggcctgaaaaccagcgaaaaatggtttcgtatgggttttcgtagcctgagcgaaattatgagcgataaaaccctgaaattcaccaagatgcagaaagcgggttttctgtattatgaagatctggttagctgtgttacccgtgccgaagccgaagcagttggtgttctggttaaagaagcagttcacgcatttctgccggatgcatttgttaccatgaccggtggttttcgtcgtggtaagaaaattggtcatgatgtggattttctgattaccagtccgggtagcgcagaagatgaagaacagctgctgccgaaagttattaatctgtgggaaaagaaaggtctgctgctgtattacgatctggttgaaagcaccttcgagaaattcaaactgccgagccgtcaggttgataccctggatcactttcagaaatgttttcttatcctgaagctgcatcatcagcgtgttgatagcagcaaaagcaatcagcaagaaggtaaaacctggaaagcaattcgtgttgatctggttctgtgtccgtatgaaaatcgtgcatttgcactgttaggttggaccggtagtcgtcagtttgaacgtgatattcgtcgttatgcaacccatgaacgtaaaatgctgctggataatcatgccctgtatgataaaaccaaacgcgtgttcctgaaagccgaaagcgaagaagaaatttttgcacatctgggccttgattacattgaaccgtgggaacgtaatgca

SEQ ID NO: 63 - DNA, 1167 bp, synthetic construct
  source 1..1167: mol_type = other DNA
atgggtcatcagctggttgttcgtaccgattatagcgcaaccccgaatccgggttttcagaaaacaccgcctctggcagttaaaaagattagccagtatgcatgtcagcgtaaaaccacgctgaataactacaacaaaatcttcaccgatgcctttgaaattctggcagaaaacgccgaatttaaagaaaacgaagttagctacgtgacctttaaacgtgcagcaagcgttctgaaaagcctgccgtttaccattaaaagcatgaaagataccgaaggtattccgtgtctgggtgataaagtgaaaaagatcatcgaagaaatcatcgaggatggtgaaagcagcgaagttaaagcagttctgaatgatgaacgttaccagagcttcaaactgtttaccagcgtttttggtgttggcctgaaaaccagcgaaaaatggtttcgtatgggttttcgtagcctgagcgaaattctgagcgataaaaccctgaaattcaccaaaatgcagaaagccggtttcctgtattatgaagatctggttagctgtgttacccgtgccgaagccgaagcagttggtgaactggttaaagaagcagttcacgcatttctgccggatgcatttgttaccattaccggtggttttcgtcgtggtaagaaaattggtcatgatgtggattttctgattaccagtccgggtagcgaagaagatgaagaacagctgctgccgaaagttattaatctgtgggaaaagaaaggtctgctgctgtatagcgatctggttgaaagcacctttgagaaattcaaactgccgagccgtcaggttgataccctggatcactttcagaaatgttttcttatcctgaagctgcatcatcagcgtgttgatagcagcaaaagcaatcagcaagaaggtaaaacctggaaagcaattcgtgttgatctggtggtttgtccgtatgaacgtcgtgcatttgcactgttaggttggaccggtagtcgtcagtttgaacgtgatattcgtcgttatgcaacccatgaacgtaaaatgctgctggataatcatgccctgtatgataaaaccaaacgcgtgttcctgaaagccgaaagtgaagaagaaatttttgcccatctgggccttgattacattgaaccgtgggaacgtaatgca

SEQ ID NO: 64 - DNA, 1167 bp, synthetic construct
  source 1..1167: mol_type = other DNA
atgggtcatcagctggttgttcgtaccgattatagcgcaaccccgaatccgggttttcagaaaacaccgcctctggcagttaaaaagattagccagtatgcatgtcagcgtaaaaccacgctgaataactacaacaaaatcttcaccgatgcctttgaaattctggcagaaaacgccgaatttaaagaaaacgaagttagctacgtgacctttatgcgtgcagcaagcgttctgaaaagcctgccgtttaccattaaaagcatgaaagataccgaaggtattccgtgtctgggtgataaagtgaaaaagatcatcgaagaaatcatcgaggatggtgaaagcagcgaagttaaagcagttctgaatgatgaacgttaccagagcttcaaactgtttaccagcgtttttggtgttggcctgaaaaccagcgaaaaatggtttcgtatgggttttcgtagcctgagcgatattatgagcgataaaaccctgaaattcaccaagatgcagaaagcgggttttctgtattatgaagatctggttagctgtgttacccgtgccgaagccgaagcagttggtgttctggttaaagaagcagttcacgcatttctgccggatgcatttgttaccatgaccggtggttttcgtcgtggtaagaaaattggtcatgatgtggattttctgattaccagtccgggtagcgcagaagatgaagaacagctgctgccgaaagttattaatctgtgggaaaagaaaggtctgctgctgtattacgatctggttgaaagcaccttcgagaaattcaaactgccgagccgtcaggttgataccctggatcactttcagaaatgttttcttatcctgaagctgcatcatcagcgtgttgatagcagcaaaagcaatcagcaagaaggtaaaacctggaaagcaattcgtgttgatctggttctgtgtccgtatgaaaatcgtgcatttgcactgttaggttggaccggtagtcgtcagtttgaacgtgatattcgtcgttatgcaacccatgaacgtaaaatgctgctggataatcatgccctgtatgataaaaccaaacgcgtgttcctgaaagccgaaagcgaagaagaaatttttgcacatctgggccttgattacattgaaccgtgggaacgtaatgca

SEQ ID NO: 65 - DNA, 1167 bp, synthetic construct
  source 1..1167: mol_type = other DNA
atgggtcatcagctggttgttcgtaccgattatagcgcaaccccgaatccgggttttcagaaaacaccgcctctggcagttaaaaagattagccagtatgcatgtcagcgtaaaaccacgctgaataactataaccacattttcaccgatgcctttgaaattctggcagaaaacgccgaatataaagaaaacgaagttagctacgtgacctttatgcgtgcagcaagcgttctgaaaagcctgccgtttaccattattagcatgaaagataccgaaggtattccgtgtctgggcgataaaatcaaatgcatcattgaagagattcttgaggatggtgaaagcagcgaagttaaagcagttctgaatgatgaacgttaccagagcttcaaactgtttaccagcgtttttggtgttggcctgaaaaccgcagaaaaatggtatcgtatgggttatcgtagcctgagcaaaatcatgagcgataaaaccctgaaattcaccaaaatgcagaaagccggtttcctgtattatgaagatctggttagctgtgttacccgtgccgaagccgaagcagttggtgttctggttaaagaagcagttcacgcatttctgccggatgcgtttgttaccatgaccggtggttttcgtcgtggtaagaaaattggtcatgatgtggattttctgattaccagtccgggtagcgcagaagatgaagaacagctgctgccgaaagttattaatctgtgggaaaagaaaggtctgctgctgtattacgatctggttgaaagcaccttcgagaaattcaaactgccgagccgtcaggttgataccctggatcactttcagaaatgttttcttatcctgaagctgcatcatcagcgtgttgatagcagcaaaagcaatcagcaagaaggtaaaacctggaaagcaattcgtgttgatctggtgatgtgtccgtatgaaaatcgtgcatttgcactgttaggttggaccggtagtcgtcagtttgaacgtgatattcgtcgttatgcaacccatgaacgtaaaatgctgctggataatcatgccctgtatgataaaaccaaacgcgtgttcctgaaagccgaaagcgaagaagaaatttttgcacatctgggccttgattacattgaaccgtgggaacgtaatgca

SEQ ID NO: 66 - DNA, 1167 bp, synthetic construct
  source 1..1167: mol_type = other DNA
atgggtcatcagctggttgttcgtaccgattatagcgcaaccccgaatccgggttttcagaaaacaccgcctctggcagttaaaaagattagccagtatgcatgtcagcgtaaaaccacgctgaataactataaccacattttcaccgatgcctttgaaattctggccgaaaactatgagttcaaagaaaacgaagttagctatgtgacctttatgcgtgcagcaagcgttctgaaaagcctgccgtttaccattattagcatgaaagataccgaaggtctgccgtgtctgggtgataaagttaaatgcattatcgaagagatcatcgaagatggtgaaagcagcgaagttaaagcagttctgaatgatgaacgttaccagagcttcaaactgtttaccagcgtttttggtgttggcctgaaaaccagcgaaaaatggtttcgtatgggttttcgtagcctgagcaaaatcatgagcgataaaaccctgaaattcaccaaaatgcagaaagccggtttcctgtattatgaagatctggttagctgtgttacccgtgccgaagccgaagcagttggtgttctggttaaagaagcagtttgggcatttctgccggatgcatttgttaccatgaccggtggttttcgtcgtggtaagaaaattggtcatgatgtggattttctgattaccagtccgggtagcgcagaagatgaagaacagctgctgccgaaagttattaatctgtgggaaaagaaaggtctgctgctgtattacgatctggttgaaagcaccttcgagaaattcaaactgccgagccgtcaggttgataccctggatcactttcagaaatgttttcttatcctgaagctgcatcatcagcgtgttgatagcagcaaaagcaatcagcaagaaggtaaaacctggaaagcaattcgtgttgatctggtgatgtgtccgtatgaaaattatgcatttgcactgttaggttggaccggtagtcgtcagtttgaacgtgatctgcgtcgttatgcaacccatgaacgtaaaatgatgctggataatcatgccctgtacgataaaacgaaacgcgtgttcctgaaagccgaaagcgaagaagaaatttttgcacatctgggccttgattacattgaaccgtgggaacgtaatgca

SEQ ID NO: 67 - DNA, 1167 bp, synthetic construct
  source 1..1167: mol_type = other DNA
atgggtcatcagctggttgttcgtaccgattatagcgcaaccccgaatccgggttttcagaaaacaccgcctctggcagttaaaaagattagccagtatgcatgtcagcgtaaaaccacgctgaataactataaccacatttttaccgatgcgctggaaattctggcagaatattcggaatttaaagaaaacgaggtgagctacgttacctttatgcgtgcagcaagcgttctgaaaagcctgccgtttaccattattagcatgaaagataccgaaggtattccgtgtctgggtgataaagtgaaatgcatcattgaagagattctggaagatggtgaaagcagcgaagttaaagcagttctgaatgatgaacgttaccagagcttcaaactgtttaccagcgtttttggtgttggcctgaaaaccgcagaaaaatggtttcgtatgggttatcgtagcctgagcaaaatcatgagcgataaaaccctgaaattcaccaaaatgcagaaagccggtttcctgtattatgaagatctggttagctgtgttacccgtgccgaagccgaagcagttggtgttctggttaaagaagcagtttgggcatttctgccggatgcatttgttaccatggttggtggttttcgtcgtggtaagaaaattggtcatgatgtggattttctgattaccagtccgggtagcgcagaggatctggaacagctgctgccgaaagttattaatctgctggaaaagaaaggtctgctgctgtattacgatctggttgaaagcaccttcgagaaattcaaactgccgagccgtcaggttgataccctggatcactttcagaaatgttttcttatcctgaagctgcatcatcagcgtgttgatagcagcaaaagcaatcagcaagaaggtaaaacctggaaagccgttcgtgttgatctggtgatgtgtccgtatgaaaatcgtgcatttgcactgttaggttggaccggtagtcgtcagtttgaacgtgatattcgtcgttatgcaacccatgaacgtaaaatgctgctggataatcatgccctgtatgataaaaccaaacgcgtgttcctgaaagccgaaagcgaagaagaaatttttgcacatctgggccttgattacattgaaccgtgggaacgtaatgca

SEQ ID NO: 68 - DNA, 1167 bp, synthetic construct
  source 1..1167: mol_type = other DNA
atgggtcatcagctggttgttcgtaccgattatagcgcaaccccgaatccgggttttcagaaaacaccgcctctggcagttaaaaagattagccagtatgcatgtcagcgtaaaaccacgctgaataactataaccacaaatttaccgatgcgctggaaattctggcagaatattcggaatttaaagaaaacgaggtgagctacgttacctttatgcgtgcagcaagcgttctgaaaagcctgccgtttaccattattagcatgaaagataccgaaggtattccgtgtctgggcgataaaatcaaatgtctgattgaagagattcttgaggatggtgaaagcagcgaagttaaagccattaaaaacgatgaacgttaccagacgctgaaactgtttaccagcgtttttggtgttggcctgaaaaccgcaaagaaatggtatcgtatgggttatcgtagcctgagcaaagttatgagcgataaaaccctgaaattcaccaaaatgcagaaagccggtttcctgtattatgaagatctggttagtccggttacacgtgccgaagccgaagcagttggtgttattgttaaagaagcagtttgggcatttctgccggatgcatttgttaccatggttggtggttttcgtcgtggtaagaaaattggtcatgatgtggattttctgattaccagtccgggtagcgcagaggatctggaacagctgctgccgaaagttattaatctgctggaaaagaaaggtctgctgctgtattacgatctggttgaaagcaccttcgagaaattcaaactgccgagccgtcaggttgataccctggatcactttcagaaatgctttcttatcattaaactgccgcatcagtgggttgatagcagcaaaagcaatcagcaagaaggtaaaacctggaaagccgttcgtgttgatctggttctggcaccgtatgaaaatcgtgcatttgcactgttaggttggaccggtagtcgtcagtttgaacgtgatattcgtcgttatgcaacccatgaacgtaaaatgctgctggataatcatcgtctgtacgataaaacgaaacgcgtgttcctgaaagccgaaagcgaagaagaaatttttgcacatctgggccttgattatgttgaaccgtgggaacgtaatgca

SEQ ID NO: 69 - DNA, 1167 bp, synthetic construct
  source 1..1167: mol_type = other DNA
atgggtcatcagctggttgttcgtaccgattatagcgcaaccccgaatccgggttttcagaaaacaccgcctctggcagttaaaaagattagccagtatgcatgtcagcgtaaaaccacgctgaataacaaaaaccacaaatttaccgatgcgctggaaattctggcagaatattcggaatataaagaaaacgaggtgagctacgttacctttatgcgtgcagcaagcgttctgaaaagcctgccgtttaccattattagcatgaaagatctggaaggtattccgtgtctgggcgataaaatcaaatgtctgattgaagagattctggaaaacggctatagcagcgaagttaaagccatcaaaaatgatgaacgttaccagacgctgaaactgtttaccagcgtttttggtgttggcctgaaaaccgcaaagaaatggtatcgtaaaggttatcgtagcctgagcgaactgatgagcgataaaaccctgaaatttaccaaaatgcagaaggcaggcttcaaatattacgaagatctggttagtccggttacacgtgccgaagccgaagcaattggtgttattgttaaagaagcagttcacgcatttctgccggatgccgaagttaccatggttggtggttttcgtcgtggtaagaaaattggtcatgatgtggattttctgattaccagtccgggtagcgcagaggatctggaacagctgctgccgaaagttgttaatctgctggaagaaaaaggtctgctgctgtattatgatctggttgaaagcaccttcgagaaattcaaactgccgagccgtcaggttgataccctggatcattttgccaaatgcttcatgatcattaaactgccgcatcagtgggttgatccgagcaaaagcaatcagcaagaaggtaaaacctggaaagcagttcgtgttgatctggtgctggcaccgtatgaaaatcgtgcatttgcactgttaggttggaccggtagtcgtcagtttgaacgtgatattcgtcgttatgcaacccacgagaaaaatatgggcttagataatcaccgcctgtacgataaaacaaaacgcgtgtttctgaaagccgaaagcgaagaagaaatttttgcacatttaggcctggattatgttgaaccgtgggaacgtaatgca

SEQ ID NO: 70 - DNA, 1167 bp, synthetic construct
  source 1..1167: mol_type = other DNA
atgggtcatcagctggttgttcgtaccgattatagcgcaaccccgaatccgggttttcagaaaacaccgcctctggcagttaaaccgctgagccagtatgcatgtcagcgtcgtaccacactgcagaataataacaaaaagtttaccgatgcgctggaagttctggcagaatatgaagaatataaagaaaacgaggtgagcaaggtgacctttgaacgtgcagcaagcgttctgaaaagcctgccgaaagaaatcaaaagcctgaaagatattgaaggcattccgtgtctgggtgacaaaaccaaaaagatcatcgaagaaattctggaaaacggctatagcaaagaggtggaaaagatcaaaaaggatgaacgttatcaggccctgaaactgtttaccagcgtttttggtgttggcctgaaaaccgcaaagaaatggtatgaaaaaggttatcgtaccctggaagaggtgaagaaagataagaatctgaagtacaccaaaatgcagaaaagcggtctggaatattatgaggatctgaataaaccggtgtcacgtgcagaagcagaagccgttgagaaaattgttaaagaagccgtgaaaaagtatctgccgaatgcaattgtgaccagcgttggtggttttcgtcgtggtaaaaagattggtcatgatgtggatattctgatcaccacaccggaagaagaaaacaaactgaaagaactgctgaagaaggtggtcgaatatctggaagaaaaaggtctgctgctgtataaagatctggttgaaagcaccttcgagaaattcaaactgccgagccgtcaggttgataccctggatcattttgataaatgcttcatgatcatcaaactgtatgatgccgatgttgatccgagcctgagtcagtataatgaaaagaaagattggcgtgccgttcgtgttgatctggttattgcaccgtatgatgtttatgcatttgcactgttaggttggaccggtagtcgtcagtttgaacgcgatattcgtcgttatgcaacccatgagaaaaatatgctgctggataatcacagcctgtatgatattaccaaccgcaaatttctggaagccaaaagcgaagaagagatctttaaacatctgggccttgaatatgtggaaccgagcgaacgtaatgca

SEQ ID NO: 71 - DNA, 1167 bp, synthetic construct
  source 1..1167: mol_type = other DNA
atgggtcatcagctggttgttcgtaccgattatagcgcaaccccgaatccgggttttcagaaaacaccgcctctggcagttgaaccggttagccagtatgcatgtcagcgtcgtaccacactggataacaaaaacaaaaagtttaccgacgcctttgaaaccctggcagaatatgccgaatataaagaaaacgaagtgagcaaagtgacctttgaacgtgcagcaagcgttctgaaaagcctgccgaaagaaatcaaaagcctgaaagatattgaaggcattccgtgtctgggtgacaaaagcaagaaactgattgaagaaattctggaaaacggctacagcaaagaagtggaaaagatcaaaaaggatgagcgctaccagaaactgaaactgtttaccagcgtttttggtgttggcctgaaaaccgcaaataaatggattgaaaaaggctaccgtaagcttgaggatgtgatcaatgataaaaacctgaagctgaccaagatgcagaaagaaggtctgaaatattacgaggatctgaccaaaccggtgtcacgtgcagaagcagaagccgttaaaaagattgttgaagaagccgtgtataagtatctgccgaatgcaaaagttaccctgtgtggtggttttcgtcgtggtaagaaaattggtcatgatgtggatattctgatcaccagtccggaagatgagaagaagctgaaagaactgctggaaaaagtggtgaaatacctggaagaaaaaggcctgctgctgtatcatgatctggttgaaagcaccttcgagaaattcaaactgccgagccgtcaggttgataccctggatcattttgccaaatgcttcatgatcatcaaactgtattatagcgaagtggatccgagcattagcgataccattgaaggtaaacaatggcgtgcagttcgtgttgatctggtgattgcaccgtatgatcagtatgcctttgcactgttaggttggaccggtagtcgtcagtttgaacgcgatattcgtcgttatgcaacccatgagaaaaatatggccctggataatcatggtctgtatgatctgacccgtcgtgaacgtctggaagccaaaagcgaagaagaaatctttaaacatctgggccttgaatatgttgaaccgaccgaacgtaatgca

SEQ ID NO: 72 - DNA, 1167 bp, synthetic construct
  source 1..1167: mol_type = other DNA
atgggtcatcagctggttgttcgtaccgattatagcgcaaccccgaatccgggttttcagaaaacaccgcctctggcagttgagaaaatttcacagtatgcatgtcagcgtaaaaccacactggataatcgcaacaaaaagtttaccgatgcctttgaagttctggccgaatatgaagagtataaagaaaacgaagtgagcaaggtgacctttgaacgtgcagcaagcgttctgaaaagcctgccgtatgaaatcaaaagcatcaaagatattgatggcattccgtgcctgggtgacaaaaacaaaaagatcattgaagaaatcctggaaaacggctatagcaaagaagtggaaaaactgaaaaaggatgaacgttatcaggccctgaaactgtttaccagcgtttttggtgttggcctgaaaaccgcaaataaatggtatgaaaaaggttaccgtacgcttgaggatgtgatcaatgataaaaatctgaaactgaccaaaatgcagaaaatcggcatcaaatattacgaggatctgagcaaaccggtgtcacgtgccgaagccgaagcagttatgaaaattgttaaagaagccgtgcacaagtttctgccgaatgcaaaagttaccatggttggtggttttcgtcgtggtaaaaagattggtcatgatgtggatattctgattaccgcaccggaaaatgaagagaaactgaaagaactgctggaaaaggtggtgaaatatctggaagaacagggtctgctgctgtataaagatctggttgaaagcaccttcgagaaattcaaactgccgagccgtcaggttgataccctggatcattttagcaaatgctttatgatcatcaaactggacctggaagaagttgatccgagcattagcccgagcattgaaggtaaaaagtggcgtgcagttcgtgttgatctggttattgcaccgtatgatgaatatgcatttgcactgttaggttggaccggtagtcgtcagtttgaacgcgatattcgtcgttatgcaacccatgagaaaaatatgctgctggataaccatggtctgtatgatctgaccacacgtaaacgtctggaagccaaaagcgaagaagaaatctttaaacatctgggccttgaatacgtggaaccgaaagaacgtaatgca

SEQ ID NO: 73 - DNA, 1167 bp, synthetic construct
  source 1..1167: mol_type = other DNA
atgggtcatcagctggttgttcgtaccgattatagcgcaaccccgaatccgggttttcagaaaacaccgcctctggcagttgagaaaatttcacagtatgcatgtcagcgtaaaaccacgctggataacaaaaacaaaaagttcaccgatgcctatgaagtgctggcagaatatgccgaatataaagaaaacgaagtgagcaaagtgacctttgaacgtgcagcaagcgttctgaaaagcctgccgaaagaaatcaaaagcatcgaagatctgaaaggtattccgtgtctgggtgataaaaccaaaaagctgattgaagagattctggaaaacggcaaaagcaaagaagtggaaaagatcaaaaaggatgagcgctatcagatcctgaaactgtttaccagcgtttttggtgttggcctgaaaaccgcaaataaatggtataacaaaggttaccgtacgcttgaggatgtgatcaatgataaaaatctgaaactgaccaaaatgcagaaaagcggcatcaaatactatgaggatctgaataaaccggttagccgtgcagaagcagaagccgttaccaaaattgttaaagaagccgtgtataagtttctgccgaatgcacaggttaccctggttggtggttttcgtcgtggtaaaaagattggtcatgatgtggatattctgattaccacaccgtccaaagaagaagaactgaaagaactgctggaaaaggtggtgaaatatctggaagaacgtggtctgctgctgtataaagatctggttgaaagcaccttcgagaaattcaaactgccgagccgtcaggttgataccctggatcattttgccaaatgcttcatgatcattaaactgccgctggaatatgttgatccgaaagtcagcaaatatatcgagggtaaaaagtggcgtgcagttcgtgttgatctggttattgcaccgtatgatcgttttgcatttgcactgttaggttggaccggtagtcgtcagtttgaacgcgatattcgtcgttatgcaacccatgagaaaaatatgctgctggataatcacagcctgtatgatctgaccagccgtaaatacctggaagccaaaagtgaagaagagatctttaaacatctgggccttgaatatgtggaaccggaagaacgcaatgca

SEQ ID NO: 74 - DNA, 1167 bp, synthetic construct
  source 1..1167: mol_type = other DNA
atgggtcatcagctggttgttcgtaccgattatagcgcaaccccgaatccgggttttcagaaaacaccgcctctggcagttaaaccgattagccagtatgcatgtcagcgtcgtaccacactggaaaacaaaaatgaaaaattcaccgatgcctttgaagtgctggcagaatatgccgaatataaagaaaacgaagtgagcaaagtgacctttgaacgtgcagcaagcgttctgaaaagcctgccgaaagaaatcaaaagcatcgaagatctgaaaggtattccgtgtctgggtgacaaaattaagaaagagattgaagaaatcctggaaaacggctatagcaaagaagtggaaaagatcaaaaaggatgaacgctaccagacctataaactgtttaccagcgtttttggtgttggcctgaaaaccgcaaagaaatggtatgaaaaaggttatcgtaccctggaagaagtgatcaacgataaaaacctgaagttcaccaagatgcagaaaaacggcatcaaatactatgaggatctgaaacgtgatgttacccgtgcagaagcagaagccgttctgggtattgttcgtgaagccgttaaacgttttctgccgaatgccgaagttaccctggttggtggttttcgtcgtggtaaaaagattggtcatgatgtggatgttctgattaccacaccggaagaggaatcaaaactgcatgaactgctgcctaaagttctggcatatctggaagaacagggtctgctgctgtattatgatctggttgaaagcaccttcgagaaattcaaactgccgagccgtcaggttgataccctggatcattttatgaaatgctttaccattatcaagctgccggtggaaaaagttgatccgagcctgagtccgacactggaaggtaaaaagtggcgtgcagttcgtgttgatctggtgctggcaccgtgggaatatcgtgcatttgcactgttaggttggaccggtagtcgtcagtttgaacgcgatattcgtcgttatgcaacccatgaacgtaatatgctgctggataatcatctgctgtatgatcgtaccgaacgtcgttttctggaagcacgtagcgaagaagaaatttttcgtcatctgggccttgaatatgttgaaccggcagaacgtaatgca

SEQ ID NO: 75 - DNA, 1167 bp, synthetic construct
  source 1..1167: mol_type = other DNA
atgggtcatcagctggttgttcgtaccgattatagcgcaaccccgaatccgggttttcagaaaacaccgcctctggcagttaaaccgattagccagtatgcatgtcagcgtcgtaccacactggataacaaaaatcgtgaatttaccgatgcctttgaagtgctggcagaatatgccgaatataaagaaaacgaagtgagcaaagtgacctttgaacgtgcagcaagcgttctgaaaagcctgccgcatcgtattaatagcatggaagatattgaaggtattccgtgcctgggtgacaaaattaagaaactgattgaagaaatcctggaaaacggcaccagcaaagaagttgagaaaatcaaaaaggatgagcgctaccagaacctgaaactgtttaccagcgtttttggtgttggcctgaaaaccgcaaagaaatggattgaaaaaggttatcgtaccctggaagaagtgatcaacgataaaaacctgaagttcaccaaaatgcagaaagccggtatcaaatactatgaagatctgacccgtgaagttacccgtgcagaagcagaagccgttctgggtattgttcgtgaagcagttcaccagtttctgccgaatgcaaccgttacactggttggtggttttcgtcgtggtaaaaagattggtcatgatgtggatgttctgattaccagtccggaagaagaaggtaaactgcgtagcctgctgccgaaagttgttgaactgctggaagaacgtggtctgctgctgtattatgatctggttgaaagcaccttcgagaaattcaaactgccgagccgtcaggttgataccctggatcactttcagaaatgctttcttatcattaaactgccggattttctggtggatccgagcaaaagcggtaaacgtgaaggtaaaaagtggcgtgcagttcgtgttgatctggtgctggcaccgtatgaacgtcgtgcatttgcactgttaggttggaccggtagtcgtcagtttgaacgcgatattcgtcgttatgcaacccatgaacgtaatatgctgctggataatcatagcctgtatgataccaccaaacgcaaatttctgcctgcggaaagcgaagaagaaatctttaaacatctgggccttgaatatgtggaaccgcaagaacgtaatgca

SEQ ID NO: 76 - DNA, 1167 bp, synthetic construct
  source 1..1167: mol_type = other DNA
atgggtcatcagctggttgttcgtaccgattatagcgcaaccccgaatccgggttttcagaaaacaccgcctctggcagttaaaaagattagccagtatgcatgtcagcgtaaaaccacgctgaataactataaccgcatttttaccgatgcctttgaaatcctggcagaatatgccgaatttaaagaaaacgaagtgagcaacgtgacctttaaacgtgcagcaagcgttctgaaaagcctgccgtatcgtattaccagcatggaagataccgaaggtattccgtgtctgggtgataaagttaaaggtctgattgaagagatcatcgaaaatggcaccagcaaagaagtggaaaagatcaaaaatgatgagcgctaccagaccttcaaactgtttaccagcgtttttggtgttggcctgaaaaccgcagaaaaatggtatgaacgtggttatcgtaccctggaagaagtgattagcgataaaaccctgaaattcaccaaaatgcagaaagcaggtctgctgtattatgaagatctgacccgttgtgttacccgtgcagaagcagaagccgttctggttctggtgcgtgaagcagtttggagctttctgccggatgcaaatgttaccatgaccggtggttttcgtcgtggtaagaaaattggtcatgatgtggattttctgattaccagtccgggtgaagaaggtaaactggaaagcctgctgccgaaagttgttaccctgctggaagaacgtggtctgctgctgtactacgatctggttgaaagcacctttgagaaattcaaactgccgagccgtcaggttgataccctggatcactttcagaagtgctttctgattgtcaaactggaacatcagcgtgttgatagcagcaaaagcgaacatcgtgaaggtaaagattggcgtgcaattcgtgttgatctggtggttgcaccgtatgaacgccgtgcatttgcactgttaggttggaccggtagtcgtcagtttgaacgtgatattcgtcgttatgcaacccatgaacgtaacatgattctggataatcaccgtctgtatgatcgtaccaaacgtcagtttctgaaagccgaaagcgaagaagaaatttttgcacatctgggccttgattatgttgaaccgagcgaacgtaatgca

SEQ ID NO: 77 - DNA, 1167 bp, synthetic construct
  source 1..1167: mol_type = other DNA
atgggtcatcagctggttgttcgtaccgattatagcgcaaccccgaatccgggttttcagaaaacaccgcctctggcagttaaaccgattagccagtatgcatgtcagcgtcgtaccacactggataacaaaaactataaattcaccgatgcctttgaagtgctggcagaatatgccgaatataaagaaaacgaagtgagcaaagtgacctttgaacgtgcagcaagcgttctgaaaagcctgccgtatgaaatcaaaagcatcgaagatctgaaaggtattccgtgtctgggtgacaaaattaagaaactgattgaagaaatcctggaaaacggctatagcaaagaagtggaaaagatcaaaaaggatgaacgctaccagacctataaactgtttaccagcgtttttggtgttggcctgaaaaccgcaaagaaatggtatgaaaaaggttatcgtaccctggaagaagtgatcaacgataaaaacctgaagttcaccaagatgcagaaaaacggcatcaaatactatgaggatctgaaacgtgatgttagccgtgcagaagcagaagccgttctgaccattgttcgtgaagcagttcgtcgttttctgccgaatgccgaagttaccctggttggtggttttcgtcgtggtaaaaagattggtcatgatgtggatgttctgattaccagtccggaagaggaatcaaaactgcgtgaactgctgccgaaagttgttgcatatctggaagaacagggtctgctgctgtattatgatctggttgaaagcaccttcgagaaattcaaactgccgagccgtcaggttgataccctggatcattttcgtaaatgctttatgattatcaagctgccggttgattgggttgatccgagcctgagtccgtttctggaaggtaaaaagtggcgtgcagttcgtgttgatctggtgctggttccgcatgaagcacgtgcatttgcactgttaggttggaccggtagtcgtcagtttgaacgcgatattcgtcgttatgcaacccatgaacgtgatatgctgctggataatcattggctgtatgatcgtaccgcacgtcgctttttaccggcagaaagcgaagaagaaatttttcgtcatctgggtctgccttatgttgaacctgcagaacgtaatgca

SEQ ID NO: 78 - DNA, 1167 bp, synthetic construct
  source 1..1167: mol_type = other DNA
atgggtcatcagctggttgttcgtaccgattatagcgcaaccccgaatccgggttttcagaaaacaccgcctctggcagttaaaccgattagccagtatgcatgtcagcgtcgtaccacactggaaaacaaaaacaagaaatttaccgatgcctttgaagtgctggcagaatatgccgaatataaagaaaacgaagtgagcaaagtgacctttgaacgtgcagcaagcgttctgaaaagcctgccgtatgaaatcaaaagcatcgaagattgtaaaggcattccgtgtctgggtgataaaattctgaaactgattgaagaaatcctggaaaacggctatagcgaagaagtgaaaaagatcgaaaaagatgaacgctaccagacctataaactgtttaccagcgtttttggtgttggcctgaaaaccgcaaagaaatggtatgaaaaaggtattcgtaccctggaagagtacatcaacaacaaaaatctgaagctgaccaaaatgcagaagtacggcatcaaatattacgaggatctgaataaaccggttacacgtgcagaagcagaagcaattctggaaattgttaaagaagccgtgaaaaagtatctgccggatgccgaagttacccaggttggtggttttcgtcgtggtaaaaagattggtcatgatgtggatgttctgattaccagtccgagtgatgaaagcaaactgaaagaactgctggaaaaagtggtgaaagatctggaagaaaaaggtctgctgctgtattatgatctggttgaaagcaccttcgagaaattcaaactgccgagccgtcaggttgataccctggatcattttgccaaatgcttcatgatcatcaaactgtacctggaaaaggttgatccgaaactgagcaaaaacatcgagaaaaagaaatggcgtgcagttcgtgttgatctggtggttgcaccgtatgattataaagcctttgcactgttaggttggaccggtagtcgtcagtttgaacgcgatattcgtcgttatgcaacccatgagaaaaatatgctgctggataatcatggcctgtatgataccacacagcgcaaatttctggaagccaaaagtgaagaagaaatctttcagcatctgggccttgaatatgttgaaccggcagaacgtaatgca

SEQ ID NO: 79 - DNA, 1167 bp, synthetic construct
  source 1..1167: mol_type = other DNA
atgggtcatcagctggttgttcgtaccgattatagcgcaaccccgaatccgggttttcagaaaacaccgcctctggcagttaaaccgattagccagtatgcatgtcagcgtcgtaccacactggataacaaaaacaaaaagtttaccgatgcctttgaagtgctggccgaatattatgagtataaagaaaacgaggtgtccaaagtgacctttaaacgtgcagcaagcgttctgaaaagcctgccgaaagaaatcaaaagctttgaagatgtgaaaggcattccgtgtctgggtgataaaaatcgcaaactgattgaagagattctggaaaacggttatagcgaagaggtgaaaaagatcgaaaaagatgaacgctatcaggcctataaactgtttaccagcgtttttggtgttggcctgaaaaccgcaaagaaatgggttgaaaaaggttatcgtaccctggaagagtacatcaacgataaaaacctgaaactgaccaagatgcagaaatgcggcatcaaatattacgaggatctgaaagcaccggttacacgtgcagaagcagaagcaattctgaaaattgttaaagaagccgtgaaaaagtatctgccggatgccgaagttaccctggttggtggttttcgtcgtggtaaaaagattggtcatgatgtggatgttctgattaccagtccgagtgatgaaagcaaactgaaagaactgctgaagaaagtggtgaaagatctggaagaaaaaggtctgctgctgtattatgatctggtggaaagcaccttcgagaaattcaaactgccgagccgtcaggttgataccctggatcattttgccaaatgcttcatgatcatcaaacttccgattgatatggtggatccgaaactgagcgaatatatcgaagagaaaaagtggcgtgcacgtcgtgttgatctggttctggcaccgtatgatcgtaaagcctttgcactgttaggttggaccggtagtcgtcagtttgaacgtgatattcgtcgttatgcaacccacgagaaaaatatgctgctggataatcatcgtctgtatgataccacacagcgcaaatttctggaagccaaaagcgaagaagaaatctttgaacatctgggccttgaatatgttgaaccgagcgaacgtaatgca

SEQ ID NO: 80 - DNA, 1167 bp, synthetic construct
  source 1..1167: mol_type = other DNA
atgggtcatcagctggttgttcgtaccgattatagcgcaaccccgaatccgggttttcagaaaacaccgcctctggcagttgagaaaatttcacagtatgcctgcaaacgtaaaaccacgctgaaaaactacaacaagaaattcaccgatgcctttgaaattctggcagaaaacgccgaatataaagaaaacgaagttagctacgtgacctataaacgtgcagcaagcgttctgaaaagcctgccgtttaccattattagcatggaagataccgaaggtattccgtgtctgggtgataaaatcaaaaagatcatcagcgagatcatcaaagatggctatagcagcgaagttgaaaaagtgctgaataacgaagagtataaaagcttcaaactgtttaccagcgtttttggtgttggcctgaaaaccgcaaagaaactgtttgaaaaaggttatcgtaccctggaagatatcatcaacgataaaagcctgaagttcaccaaaatgcagaaagcgggttttctgtattatgaggatctggttagtccggttacacgtgaagaggccgaagcagttggtgttctggttaaagaagcagttcacgcatttctgccggatgcatttgttgaaatggttggtggttttcgtcgcggtaaaaagattggtcatgatgtggattttctgatctatagcaaaggcagcgcagaaaaagaagaaaccctgctgcagaaagttattgacctgtggaaaaagaaaggcatcctgctgtattacgatctggttgaaagcaccttcgagaaattcaaactgccgagccgtcaggttgataccctggatcactttcagaagtgctttctgattctgaaactggaacatcagcgtgttgatagcagcaaaagcagccatatggaaggtaaaacctggaaagccgttcgtgttgatctggttctggcaccgtttgaaaattatgcatttgcactgttaggttggaccggtagtcgtcagtttgaacgtgatattcgtcgttatgcaacccatgaacgtaaaatgatgctggataatcaccgcctgtacgacaaagaaaaacgcgaatttctgaaagccgatagcgtggaagaaatctttaaacatctgggccttgagtatatcgaaccgcatgaacgcaatgca

SEQ ID NO: 81 - DNA, 1167 bp, synthetic construct
  source 1..1167: mol_type = other DNA
atgggtcatcagctggttgttcgtaccgattatagcgcaaccccgaatccgggttttcagaaaacaccgcctctggcagttgagaaaatttcacagtatgcctgcaaacgtaaaaccacgctgaaaaactacaacaagaaattcaccgatgcctttgaaattctggcagaaaacgccgaatataaagaaaacgaagttagctacgtgacctataaacgtgcagcaagcgttctgaaaagcctgccgtttaccattattagcatggaagataccgaaggtattccgtgtctgggtgataaaatcaaatgcatcattagcgagatcatcaacgatggttatagcagcgaagttgaaaaagtgctgaacaacgaagagtacaaaagcttcaaactgtttaccagcgtttttggtgttggcctgaaaaccgcaaagaaatggtttgaaaaaggttatcgtaccctggaagatattatcaacgacaaaagcctgaagttcaccaaaatgcagaaagcgggttttctgtattatgaggatctggttagtccggttacacgtgaagaggccgaagcagttggtgttctggttaaagaagcagttcacgcatttctgccggatgcgtttgttgaaatgaccggtggttttcgtcgtggtaaaaagattggtcatgatgtggattttctgattagcagcgcaggtagcgcagaaaaagaagaaaccctgctgcagaaagttattgacctgtggaaaaagaaaggcatcctgctgtattacgatctggttgaaagcaccttcgagaaattcaaactgccgagccgtcaggttgataccctggatcactttcagaagtgctttctgattctgaaactggaacatcagcgtgttgatagcagcaaaagcagccatatggaaggtaaaacctggaaagccgttcgtgttgatctggttctggcaccgtgggaaaattatgcatttgcactgttaggttggaccggtagtcgtcagtttgaacgtgatattcgtcgttatgcaacccatgaacgtaaaatgatgctggataatcaccgcctgtacgacaaagaaaaacgcgaatttctgaaagccgaaagcgtggaagaaatctttgaacatctgggccttgagtatattgaaccgcatgaacgcaatgca

SEQ ID NO: 82 - DNA, 1167 bp, synthetic construct
  source 1..1167: mol_type = other DNA
atgggtcatcagctggttgttcgtaccgattatagcgcaaccccgaatccgggttttcagaaaacaccgcctctggcagttaaaaagattagccagtatgcatgccagcgtaaaattaccctgaataactataaccacatcttcaccgatgcctttgaaattctggcagaaatggccgaatttaaagaaaacgaagttagctacgtgacctttatgcgtgcagcaagcgttctgaaaagcctgccgtttaccattaccagcatgaaagataccgaaggtattccgtgtctgggtgataaagtgaaatgcatcattgaagagatcatcgaagatggtgaaagcagcgaagttaaagcagttctgaatgatgaacgttaccagagcttcaaactgtttaccagcgtttttggtgttggcctgaaaaccgcagaaaaatggtttcgtatgggccatcgtagcctgagcgatattatgaaagacaaaaccatcaaatttaccaaaatgcagaaagcgggtttcctgtattatgaagatctgcgtacctgtattacccgtaccgaagccgaagcaattggtgttattgttaaagaagcagtctgggcatttgatccggatgcatttgttattatgaccggtggttttcgtcgcggtaagaaaattggtcatgatgtggattttgtgattaccagtcctggtagctgggaagatgaacgtcagctgctgccgaaagttattcgttggtgtgaaaagaaaggtcatctgctgtattacgatctggttgaaagcaccttcgagaaattcaaactgccgagccgtcaggttgataccctggatcatttccagaaatgcttcatgattctgaaactgcatttttggtggcgtgatccgagcaaaagcaatcagtgtgaaggcaaacagtggaaagcatgtcgtgttgatctggttatgtgtcattgggaacatcgtgcatttgcactgttaggttggaccggtagtcgtcagtttgaacgtgatattcgtcgttatgcaacccatgaacgtaaaatgatgctggataatcatgccctgtatgacaaaacgaaatgggtctttctgaaagccgaaagcgaagaagaaatttttcgtcatctgggtctgccgtatattgaaccgtgggaacgtaatgca

SEQ ID NO: 83 - DNA, 1167 bp, synthetic construct
  source 1..1167: mol_type = other DNA
atgggtcatcagctggttgttcgtaccgattatagcgcaaccccgaatccgggttttcagaaaacaccgcctctggcagttaaaaagattagccagtatgcatgccagcgtaaaattaccctgaataactataaccacatcttcaccgatgcctttgaaattctggcagaaatggccgaatttaaagaaaacgaagttagctacgtgacctttatgcgtgcagcaagcgttctgaaaagcctgccgtttaccattaccagcatgaaagataccgaaggtattccgtgtctgggtgataaagtgaaatgcatcattgaagagatcatcgaagatggtgaaagcagcgaagttaataaagtgctgaatgatgaacgctaccagagcttcaaactgtttaccagcgtttttggtgttggcctgaaaaccgcagaaaaatggtttcgtatgggccatcgtagcctgagcgatattctgaaagataaaaccatcaaatttaccaaaatgcagaaggcaggcttcctgtattatgaagatctgcgtagctgtattacccgtaccgaagccgaagcaattggtgttattgttaaagaagcagtctgggcatttgatccggatgcatttgttattatgaccggtggttttcgtcgcggtaagaaaattggtcatgatgtggattttgtgattaccagtcctggtagctgggaatgtgaagaacagctgctgccgaaagttattcgttggtgtgaaaagaaaggtcatctgctgtactatgatctggttgaaagcaccttcgagaaattcaaactgccgagccgtcaggttgataccctggatcatttccagaaatgcttcatgatcctgaaacatcattggtggtggcgtgatccgagcaaaagcaatcagtgtgaaggcaaacagtggaaagcatgtcgtgttgatctggtggtttgtcattgggaacatcgtgcatttgcactgttaggttggaccggtagtcgtcagtttgaacgtgatattcgtcgttatgcaacccatgaacgtaaaatgatgctggataatcatgccctgtacgacaaaaccaaatgggtatttctgaaagccgaaagcgaagaagaaatctttgaacatctgggtctgccgtatattgaaccgtgggaacgtaatgca

SEQ ID NO: 84 - DNA, 1167 bp, synthetic construct
  source 1..1167: mol_type = other DNA
atgggtcatcagctggttgttcgtaccgattatagcgcaaccccgaatccgggttttcagaaaacaccgcctctggcagttaaaaagattagccagtatgcatgccagcgtaaaattaccctgaataactataaccacatcttcaccgatgcctttgaaattctggcagaaatggccgaatttaaagaaaacgaagttagctacgtgacctttatgcgtgcagcaagcgttctgaaaagcctgccgtttaccattaccagcatgaaagataccgaaggtattccgtgtctgggtgataaagtgaaatgcatcattgaagagatcatcgaaaccggtgaaagcagcgaagttaatgcagttctgaatgatgaacgttaccagagcatgaaactgtttaccagcgtttttggtgttggcctgaaaaccgcagaaaaatggtttcgtatgggccatcgtagcctgagcgatattctgaaagataaaaccatcaaatttaccaaaatgcagaaggcaggcttcctgtattatgaagatctgcgtagctgtgttacccgtgccgaagcagatgcaattgaagttattgttaaagaagccgtctgggcatttgatccggatgcatttgttattatgaccggtggttttcgtcgcggtaagaaaattggtcatgatgtggattttgtgattaccagtcctggtagctgggaatgtgaacgtcagctgctgccgaaagttattcgttggtgtgaaaagaaaggtcatctgctgtattacgatctggttgaaagcaccttcgagaaattcaaactgccgagccgtcaggttgataccctggatcatttccagaaatgcttcatgattctgaaactgcatatgtggtgggttgatccgagcaaaagcaatcagtgtgaaggcaaacagtggaaagcaattcgtgttgatctggttatgtgtcattgggaacatcgtgcatttgcactgttaggttggaccggtagtcgtcagtttgaacgtgatattcgtcgttatgcaacccatgaacgtaaaatgatgctggataatcatgccctgtacgacaaaaccaaatgggtatttctgaaagccgaaagcgaagaagaaatctttgaacatctgggtctgccgtatattgaaccgtgggaacgtaatgca

SEQ ID NO: 85 - DNA, 1167 bp, synthetic construct
  source 1..1167: mol_type = other DNA
atgggtcatcagctggttgttcgtaccgattatagcgcaaccccgaatccgggttttcagaaaacaccgcctctggcagttaaaaagattagccagtatgcatgccagcgtaaaattaccctgaataactataaccacatcttcaccgatgcctttgaaattctggcagaaatggccgaatttaaagaaaacgaagttagccacgttacctttatgcgtgcagcaagcgttctgaaaagcctgccgtttaccattaccagcatgaaagataccgaaggtattccgtgtctgggtgataaagtgaaatgcatcattgaagagatcatcgaaaccggtgaaagcagcgaagttaagaaagttctgaatgatgaacgctaccagagcttcaaactgtttaccagcgtttttggtgttggcctgaaaaccgcagaaaaatggtatcgttggggtcatcgtagcctgagcgatattctgaaagataaaaccatcaaatttaccaaaatgcagaaggcaggcttcctgtattatgaagatctgaaacagtgtattacccgtgccgaagccgaagcaattggtgttattgttaaagaagcagtctgggcatttgatccggatgcatttgttattatgaccggtggttttcgtcgcggtaagaaaattggtcatgatgtggattttgtgattaccagtccgggtagcgcagaatgtgaacgtcgtctgctgccgaaagttattcgttggtgtgaaaagaaaggccacatgctgtattacgatctggttgaaagcaccttcgagaaattcaaactgccgagccgtcaggttgataccctggatcatttccagaaatgcttcatgattctgaaactgcatatgtggtgggttgatccgagcaaaagcaatcagtgtgaaggtaaaggttggaaagcatgtcgtgttgatctggtggtttgtcattgggaacatcgtgcatttgcactgttaggttggaccggtagtcgtcagtttgaacgtgatattcgtcgttatgcaacccatgaacgtggtatgatgctggataatcatgccctgtatgataaaacgaaatgggtctttctgaaagccgaaagcgaagaagaaatctttgaacatctgggtctgccgtatattgaaccgtgggaacgtaatgca

SEQ ID NO: 86 - DNA, 1167 bp, synthetic construct
  source 1..1167: mol_type = other DNA
atgggtcatcagctggttgttcgtaccgattatagcgcaaccccgaatccgggttttcagaaaacaccgcctctggcagttaaaaagattagccagtatgcatgccagcgtaaaattaccctgaataactataaccacatcttcaccgatgcctttgaaattctggcagaaatggccgaatttaaagaaaacgaagttagccacgttacctttatgcgtgcagcaagcgttctgaaaagcctgccgtttaccattaccagcatgaaagataccgaaggtattccgtgtctgggtgataaagtgaaatgcattattcgcgaaatcatcgaaaccggtgaaagcagcgaagttgaagcagttctgaatgatgaacgttatcaggcctttaaactgtttaccagcgtttttggtgttggcctgaaaaccgcagaaaaatggtatcgttggggttttcgtagcctgagcgatattctgaaagataaaaccctgaagttcaccaagatgcagaaagcaggttttctgtattatgaagatctgagcagctgtgttacccgtaccgaagcagaagcaattggtaaaattgttaaagaagccgtctgggcatttgatccggatgcatttgttattatgaccggtggttttcgtcgcggtaagaaaattggtcatgatgtggattttgtgattaccagtccgggtccgagcgaaatggaagaacagctgctgccgaaagtgattaattggatggaaaagaaaggccatctgctgtattacgatctggttgaaagcaccttcgagaaattcaaactgccgagccgtcaggttgataccctggatcatttccagaaatgcttcatgattctgaaactgcactattggtggcgtgatccgagcaaaagcaatcagtgtgaaggcaaacagtggaaagcaattcgtgttgatctggtggtttgtcattgggaacatcgtgcatttgcactgttaggttggaccggtagtcgtcagtttgaacgtgatattcgtcgttatgcaacccatgaacgtggtatgatgctggataatcatggtctgtatgatcgtaccaaatgggtctttctgaaagccgaaagcgaagaagaaatctttgaacatctgggtctgccgtatattgaaccgtgggaacgtaatgca

SEQ ID NO: 87 - DNA, 1167 bp, synthetic construct
  source 1..1167: mol_type = other DNA
atgggtcatcagctggttgttcgtaccgattatagcgcaaccccgaatccgggttttcagaaaacaccgcctctggcagttaaaaagattagccagtatgcatgccagcgtaaaattaccctgaataactataaccacatcttcaccgatgcctttgaaattctggcagaaatggccgaatttaaagaaaacgaagttagccacgttacctttatgcgtgcagcaagcgttctgaaaagcctgccgtttaccattaccagcatgaaagataccgaaggtattccgtgtctgggtgataaagtgaaatgcattattcgcgaaattatcgaaaccggcaccagcagcgaagttgaagcagttctgaatgatgaacgttatcaggcctttaaactgtttaccagcgtttttggtgttggcctgaaaaccgcagaaaaatggtatcgtatgggccatcgtagcctgagcgatattcgtaaagataaaagcatcaaatttaccaaaatgcagaaagccggtttcatctattatgaagatctgagcagctgtattacccgtgccgaagcagatgcaattgagaaaattgttaaagaagcctgctgggcatttgatccggatgccaaagttattatgaccggtggttttcgtcgtggtaagaaaattggtcatgatgtggattttgtgattaccagtccgggtccgagcgaaatggaacgtcagctgctgccgaaaatgattaattggtgtgaaaaacagggctatctgctgtattatgatctggttgaaagcaccttcgagaaattcaaactgccgagccgtcaggttgataccctggatcatttccagaaatgcttcatgattctgaagctgcatatgaaacgtgtggatagcagcaaaagcaatcagtgtgaaggtaaaggttggaaagcatgtcgtgttgatctggtgatgtgtcattgggaacatcgtgcatttgcactgttaggttggaccggtagtcgtcagtttgaacgtgatattcgtcgttatgcaacccatgaacgtggtatgatgctggataatcatggtctgtatgatcgtaccaaatggacctttctgaaagccgaaagcgaagaagaaatttttcgtcatctgggtctgccgtatattgaaccgtgggaacgtaatgca

SEQ ID NO: 88 - DNA, 1167 bp, synthetic construct
  source 1..1167: mol_type = other DNA
atgggtcatcagctggttgttcgtaccgattatagcgcaaccccgaatccgggttttcagaaaacaccgcctctggcagttaaaaagattagccagtatgcatgccagcgtaaaattaccctgaataactataaccacatcttcaccgatgcctttgaaattctggcagaaatggccgaatttaaagaaaacgaagttagctacgtgacctttatgcgtgcagcaagcgttctgaaaagcctgccgtttaccattaccagcatgaaagataccgaaggtattccgtgtctgggtgataaagtgaaatgcattattcgcgaaatcatcgaaaccggtcatagcagcgaagttgaagcagttctgaatgatgaacgttatcaggcctttaaactgtttaccagcgtttttggtgttggcctgaaaaccgcagaaaaatggtatcgttggggtcatcgtagcctgagcgatattcgtaaagataaaagcatcaaatttaccaaaatgcagaaagccggtttcaagtattatgaagatctgagcagccgtgttacccgtgcagaagcagaagcaattgcaaaaattgttaaagaagcaacctgggcctttgatccggatgcatttgttattatgacaggtggttttcgtcgcggtaagaaaattggtcatgatgtggattttgtgattaccagtccgggtccgagcgaaatggaacgtcgtctgctgccgtggattattaactggatgtggaaacagggtcacatgctgtattatgatctggttgaaagcaccttcgagaaattcaaactgccgagccgtcaggttgataccctggatcatttccagaaatgcttcatgattctgaagctgcatatgaaacgtgtggatagcagcaaaagcaatcagtgcgaaggtaaaaattggaaagccattcgtgttgatctggtggtttgtcattgggaacatcgtgcatttgcactgttaggttggaccggtagtcgtcagtttgaacgtgatattcgtcgttatgcaacccatgaacgtggtatgatgctggataatcatggtctgtatgatcgtaccaaacacacctttctgaaagccgaaagcgaagaagaaatctttgaacatctgggccttgagtatattgaaccgtgggaacgtaatgca

SEQ ID NO: 89 - DNA, 1167 bp, synthetic construct
  source 1..1167: mol_type = other DNA
atgggtcatcagctggttgttcgtaccgattatagcgcaaccccgaatccgggttttcagaaaacaccgcctctggcagttaaaaagattagccagtatgcatgccagcgtaaaattaccctgaataactataaccacatcttcaccgatcactttgaaattctggcagaaatggccgaattcaaagaaaatgaagttagccacgttacctttatgcgtgcagcagcagttctgaaaagcctgccgtttaccattaccagcatgaaagataccgaaggtattccgtgtctgggtgataaagtgaaacgtattattcgcgaaattatcgaaaccggcaccagcagcgaagttgaaaatgttctgaatgatgaacgctaccaggcctttaaactgtttaccagcgtttttggtgttggcctgaaaaccgcagaaaaatggtatcgttggggtcatcgtagcctgtgtgatattcgtaaagacaaaagcatcaaatttaccaaaatgcagaaggcaggcttcaaatattacgaagatctgagcagccgtattacccgtgatgaagcagaagcaattgccaaaattgttaaagaagcaacctgggcatttgatccggatgccgaagttcagatgaccggtggttttcgtcgtggtaagaaaattggtcatgatgtggattttgtgattaccagtccgggtcctgaatggatggaatggcagctgctgccgtggattattaactggatgatgaaacagggtcacatgctgtattatgatctggttgaaagcaccttcgagaaattcaaactgccgagccgtcaggttgataccctggatcatttccagaaatgcttcatgattctgaagctgcatatgaaacatgttgatccgagccagagcaatcagaatgaaggtcgtcattggaaagcatgtcgtgttgatctggtggtttgtcattgggaacatcgtgcatttgcactgttaggttggaccggtagtcgtcagtttgaacgcgatattcgtcgttatgcaacccatgaacgtggtatgatgctggataatcatggtctgtatgatcgtacccgtcatacctttctgaaagcagaaaccgaaaaagaaatctttgaacacctgggccttgagtatattgaaccgtgggaacgtaatgca

SEQ ID NO: 90 - DNA, 1167 bp, synthetic construct
  source 1..1167: mol_type = other DNA
atgggtcatcagctggttgttcgtaccgattatagcgcaaccccgaatccgggttttcagaaaacaccgcctctggcagttaaaaagattagccagtatgcatgccagcgtaaaattaccctgtgtaaccacaacaaaatcttcaccgatgcctttgaaattctggcagaaatggccgaatttaaagaaaacgaagttagctacgtgacctatatgcgtgcagcagcagttctgaaaagcctgccgtttaccattaccagcatgaaacataccgaaggtattccgtgtctgggtgataaagttaaacgcatcatcaaagagatcatcgaaaccggtcatagcagcgaagttgaaaatgttctgaatgatgaacgctaccaggcctttaaactgtttaccagcgtttttggtgttggcctgaaaaccgcagaaaaatggtatcgtatgggccatcgtagcctggaagatattcgtaaagataaaagcatcaaactgaccaaaatgcagaaagccggtttcaaatattacgatgatctgagcagccgtattacccgtgatgaagcagaagcaattgccaaaattgttaaagaagcaacctgggcatttgatccggatgcagttgttgttatgtgtggtggttttcgtcgtggtaagaaaattggtcatgatgtggattttgtgattaccagtccgggtcctgatagcatggaaatgaatctgctgccgtggatgattaactattggatgaaacagggctacatgctgtattatgatctggttgaaagcaccttcgagaaattcaaactgccgagccgtcaggttgataccctggatcactttcagaaatgtttttgcattctgatgctgcacttcaaatatcgtgatagcagccagagcgattgtcaagaaggtcagaattggaaagcatgtcgtgttgatctggtgatgtgtcattgggaacatcgtgcatttgcactgttaggttggaccggtagtcgccagtttgaacgtgatattcgtcgttatgcaacccatgaacgtggtatgatgctggataatcatggtctgtatgatcgtacccgtcatacctttctgaaggccgaaagcgaaaaagaaatctttgaacatctgggccttgagtatattgaaccgcgtgaacgtaatgca

SEQ ID NO: 91 - DNA, 1167 bp, synthetic construct
  source 1..1167: mol_type = other DNA
atgggtcatcagctggttgttcgtaccgattatagcgcaaccccgaatccgggttttcagaaaacaccgcctctggcagttaaaaagattagccagtatgcatgtcagcgtaaaaccacactgaataactgcaaccatatctttaccgatgcctttgaaattctggccgaaaactatgaatttcgcgagaatgaagttagctacctgacctttatgcgtgcagcaagcgttctgaaaagcctgccgtttaccattattagcatgaaagataccgaaggtattccgtgtctgggtgataaagtgaaatgcatcattgaagagatcatcgaagatggtgaaagcagcgaagttaaagcagttctgaatgatgaacgttaccagagcttcaaactgtttaccagcgtttttggtgttggcctgaaaaccagcgaaaaatggtttcgtatgggttttcgtagcctgagcaaaattcgtagcgataaaaccctgaaatttacccgtatgcagaaagcgggttttctgtattatgaagatctggttagctgtgttacccgtgccgaagccgaagcagttggtgttctggttaaagaagcagtttgggcatttctgccggatgcatttgttaccatgaccggtggttttcgtcgtggtaagaaaattggtcatgatgtggattttctgattaccagtccgggtagcaccgaagatgaagaacagctgctgccgaaagttattaatctgtgggaaaagaaaggtctgctgctgtattacgatctggttgaaagcaccttcgagaaattcaaactgccgagccgtcaggttgataccctggatcactttcagaaatgttttcttatcctgaagctgcatcatcagcgtgttgatagcggtaaaagcaatcagcaagaaggtaaaacctggaaagcaattcgtgttgatctggtgatgtgtccgtatgaaaatcgtgcatttgcactgttaggttggaccggtagtcgtcagtttgaacgtgatattcgtcgttatgcaacccatgaacgtaaaatgatgctggataatcatgccctgtacgataaaacgaaacgcatcttcctgaaagccgaaagcgaagaagaaatttttgcacatctgggccttgattacattgaaccgtgggaacgtaatgca

SEQ ID NO: 92 - DNA, 1167 bp, synthetic construct
  source 1..1167: mol_type = other DNA
atgcgtcatcagctggttgttcgtaccgattatagcgcaagcccgaatccgggttttcagaaaacaccgcctctggcagttaaaaagattagccagtatgcatgtcagcgtaaaaccacactgaataattgcaaccgcatttttaccgatgcctttgaagttctggccgaaaattatgaatttcgcgagaatgaagtgttttgcctggcatttatgcgtgcagcaagcgttctgaaaagcctgccgtttaccattattagcatgaaagataccgaaggtattccgtgtctgggtgataaagtgaaatgcatcattgaagagatcatcgaagatggtgaaagcagcgaagttaaagcagttctgaatgatgagcgctacaaaagcttcaaactgtttaccagcgtttttggtgttggcctgaaaaccagcgaaaaatggtttcgtatgggttttcgtaccctgagcaaaattcgtagcgataaaaccctgaaatttacccgtatgcagaaagcgggttttctgtattatgaagatctggttagctgtgttacccgtgcagaagcagaagccgttagcgttctggttaaagaagcagtttgggcatttctgccggatgcatttgttaccatgaccggtggttttcgtcgtggtaaaaagacaggtcatgatgtggattttctgattaccagtccgggtagcaccgaagatgaagaacagctgctgccgaaagttattaatctgtgggaacgtaaaggtctgctgctgtattacgatctggttgaaagcacctttgagaaactgaaactgccgagccgtaaagttgatgcactggatcactttcagaaatgttttcttatcctgaagctgcatcatcagcgtgttgatagcggtaaaagcaatcagcaagaaggtaaaacctggaaagcaattcgtgttgatctggtgatgtgtccgtatgaaaatcgtgcatttgcactgttaggttggaccggtagccgtcagtttgaacgtgatctgcgtcgttatgcaacccatgaacgtaaaatgattctggataatcacgccctgtacgataaaacgaaacgcatcttcctgaaagccgaaagcgaagaagaaatttttgcacatctgggccttgattacattgaaccgtgggaacgcaatgca

SEQ ID NO: 93 - DNA, 1167 bp, synthetic construct
  source 1..1167: mol_type = other DNA
atgcatcatctgctggttgttcgtaccgattatagcgcaaccccgaatccgggttttcagaaaacaccgcctctggcagttaaaaagattagccagtatgcatgtcagcgtaaaaccacactgaataactgcaaccatatctttaccgatgcctttgaagttctggccgaaaattatgaatttcgcgagaatgaagtgttttgcctggcatttatgcgtgcagcaagcgttctgaaaagcctgccgtttaccattattagcatgaaagataccgaaggtattccgtgtctgggtgataaagtgaaatgcattatcgaagagatcatcgaagatggtgaaagcagcgaagttaaagcagttctgaatgatgagcgctacaaaagcttcaaactgtttaccagcgtttttggtgttggcctgaaaaccagcgaaaaatggtttcgtatgggttttcgtaccctgagcaaaattcgtagcgataaaaccctgaaatttacccgtatgcagaaagcgggttttctgtattatgaagatctggttagctgtgttacccgtgcagaagcagaagccgttagcgttctggttaaagaagcagtttgggcatttctgccggatgcatttgttaccatgaccggtggttttcgtcgtggtaaaaagacaggtcatgatgtggattttctgattaccagtccgggtagcaccgaagatgaagaacagctgctgccgaaagttattaatctgtgggaacgtaaaggtctgctgctgtattacgatctggttgaaagcacctttgagaaactgaaactgccgagccgtaaagttgatgcactggatcactttcagaaatgttttcttatcctgaagctgcatcatcagcgtgttgatagcggtaaaagcaatcagcaagaaggtaaaacctggaaagcaattcgtgttgatctggtgatgtgtccgtatgaaaatcgtgcatttgcactgttaggttggaccggtagccgtcagtttgaacgtgatctgcgtcgttatgcaacccatgaacgtaaaatgattctggataatcacgccctgtacgataaaacgaaacgcatcttcctgaaagccgaaagcgaagaagaaatttttgcacatctgggccttgattacattgaaccgtgggaacgcaatgca

SEQ ID NO: 94 - DNA, 1167 bp, synthetic construct
  source 1..1167: mol_type = other DNA
atgcatcatctgctggttgttcgtaccgattatagcgcaaccccgaatccgggttttcagaaaacaccgcctctggcagttaaaaagattagccagtatgcatgtcagcgtaaaaccacactgaataactgcaaccatatctttaccgatgcctttgaaattctggccgaaaactatgaatttcgcgagaatgaaggtagctatgttgcatttatgcgtgcagcaagcgttctgaaaagcctgccgtttaccattattagcatgaaagataccgaaggtattccgtgtctgggtgataaagtgaaatgcattatcgaagagatcatcgaagatggtgaaagcagcgaagttaaagcagttctgaatgatgaacgttaccagagcttcaaactgtttaccagcgtttttggtgttggcctgaaaaccagcgaaaaatggtttcgtatgggttttcgtaccctgagcaaaattcgtagcgataaaaccctgaaatttacccgtatgcagaaagcgggttttctgtattatgaagatctggttagctgtgttacccgtgccgaagccgaagcagttggtgttctggttaaagaagcagttcgcgcatttctgccggatgcatttgttaccatgaccggtggttttcgtcgtggtaagaaaattggtcatgatgtggattttctgattaccagtccgggtagcgcagaagatgaagaacagctgctgccgaaagttattaatctgtgggaacgtaaaggtctgctgctgtattgtgatctggttgaaagcacctttgagaaactgaaactgccgagccgtaaagttgatgcactggatcactttcagaaatgttttcttatcctgaagctgcatcatcagcgtgttgatagcggtaaaagcaatcagcaagaaggtaaaacctggaaagcaattcgtgttgatctggtgatgtgtccgtatgaaaatcgtgcatttgcactgttaggttggaccggtagccgtcagtttgaacgtgatctgcgtcgttatgcaacccatgaacgtaaaatgatgctggataatcatgccctgtacgataaaacgaaacgcatcttcctgaaagccgaaagcgaagaagaaatttttgcacatctgggccttgattacattgaaccgtgggaacgcaatgca

SEQ ID NO: 95 - DNA, 1167 bp, synthetic construct
  source 1..1167: mol_type = other DNA
atgcatcatctgctggttgttcgtaccgattatagcgcaagcccgaatccgggttttcagaaaacaccgcctctggcagttaaaaagattagcccgtatgcatgtcagcgtaaaaccacactgaataactgcaaccatatctttaccgatgcctttgaagttctggccgaaaattatgaatttcgcgagaacgaaggtttctatctggcatttatgcgtgcagcaagcgttctgaaaagcctgccgtttaccattattagcatgaaagataccgaaggtattccgtgtctgggtgataaagtgaaatgcattatcgaagagatcatcgaagatggtgaaagcagcgaagttaaagcagttctgaatgatgaacgttaccagagcttcaaactgtttaccagcgtttttggtgttggcctgaaaaccagcgaaaaatggtttcgtatgggttttcgtagcctgagcaaaattcgtagcgataaaaccctgaaatttacccgcatgcagaaagcaggttttctgtattatgaagatctggttagctgtgttacccgtgcagaagcagaagccgttagcgttctggttaaagaagcagttcgcgcatttctgccggatgcatttgttaccatgaccggtggttttcgtcgtggtaagaaaattggtcatgatgtggattttctgattaccagtccgggtagcgcagaagatgaagaacagctgctgccgaaagttattaatctgtgggaacgtaaaggtctgctgctgtatagcgatctggtggaaagcacctttgaaaaactgaaactgccgagccgtaaagttgatgcactggatcactttcagaaatgttttcttatcctgaagctgcatcatcagcgtgttgatagcggtaaaagcaatcagcaagaaggtaaaacctggaaagcaattcgtgttgatctggtgatgtgtccgtatgaaaatcgtgcatttgcactgttaggttggaccggtagccgtcagtttgaacgtgatattcgtcgttatgcaacccatgaacgtaaaatgatgctggataatcatgccctgtacgataaaacgaaacgcatcttcctgaaagccgaaagcgaagaagaaatttttgcacatctgggccttgattacattgaaccgtgggaacgcaatgca

SEQ ID NO: 96 - DNA, 1167 bp, synthetic construct
  source 1..1167: mol_type = other DNA
atgcatcatcagctggttgttcgtaccgattatagcgcaagcccgaatccgggttttcagaaaacaccgcctctggcagttaaaaagattagccagtatgcatgtcagcgtaaaaccacactgaataactgcaaccatatctttaccgatgcctttgatattctggccgaaaactatgagtttaaagaaaacgaagttagctatctggcatttatgcgtgcagcaagcgttctgaaaagcctgccgtttaccattattagcatgaaagataccgaaggtattccgtgtctgggtgataaagtgaaatgcattatcgaagagatcatcgaagatggtgaaagcagcgaagttaaagcagttctgaatgatgaacgttaccagagcttcaaactgtttaccagcgtttttggtgttggcctgaaaaccagcgaaaaatggtttcgtatgggttttcgtaccctgagcaaaattcgtagcgataaaaccctgaaatttacccgtatgcagaaagcgggttttctgtattatgaagatctggttagctgtgttacccgtgccgaagccgaagcagttggtgttctggttaaagaagcagtttgggcatttctgccggatgcatttgttaccatgaccggtggttttcgtcgtggtaagaaaattggtcatgatgtggattttctgattaccagtccgggtagcaccgaagatgaagaacagctgctgccgaaagttattaatctgtgggaacgtaaaggtctgctgctgtattgtgatctggttgaaagcaccttcgagaaattcaaactgccgagccgtaaagttgatgcactggatcactttcagaaatgttttcttatcctgaagctgcatcaccagcgtgttgatagcggtaaaagcaatcagcaagaaggtaaaacctggaaagcaattcgtgttgatctggtgatgtgtccgtatgaaaatcgtgcatttgcactgttaggttggaccggtagccgtcagtttgaacgtgatctgcgtcgttatgcaacccatgaacgtaaaatgatgctggataatcatgccctgtacgataaaacgaaacgcatcttcctgaaagccgaaagcgaagaagaaatttttgcacatctgggccttgattacattgaaccgtgggaacgcaatgca

SEQ ID NO: 97 - DNA, 1167 bp, synthetic construct
  source 1..1167: mol_type = other DNA
atgcgtcatcagctggttgttcgtaccgattatagcgcaaccccgaatccgggttttcagaaaacaccgcctctggcagttaaaaagattagccagtatgcatgtcagcgtaaaaccacactgaataactgcaaccatatctttaccgatgcctttgaagttctggccgaaaattatgaatttcgcgagaacgaagtgttctacctgacctttatgcgtgcagcaagcgttctgaaaagcctgccgtttaccattattagcatgaaagataccgaaggtattccgtgtctgggtgataaagtgaaatgcatcattgaagagatcatcgaagatggtgaaagcagcgaagttaaagcagttctgaatgatgagcgctacaaaagcttcaaactgtttaccagcgtttttggtgttggcctgaaaaccagcgaaaaatggtttcgtatgggttttcgtagcctgagcaaaattcgtagcgataaaaccctgaaatttacccgtatgcagaaagcgggttttctgtattatgaagatctggttagctgtgttacccgtgccgaagccgaagcagttggtgttctggttaaagaagcagtttgggcatttctgccggatgcatttgttaccatgaccggtggttttcgtcgtggtaaaaagacaggtcatgatgtggattttctgattaccagtccgggtagcgcagaagatgaagaacagctgctgccgaaagttattaatctgtgggaacgtaaaggtctgctgctgtattgtgatctggttgaaagcacctttgagaaactgaaactgccgagccgtaaagttgatgcactggatcactttcagaaatgttttcttatcctgaagctgcatcatcagcgtgttgatagcggtaaaagcaatcagcaagaaggtaaaacctggaaagcaattcgtgttgatctggtgatgtgtccgtatgaaaatcgtgcatttgcactgttaggttggaccggtagccgtcagtttgaacgtgatctgcgtcgttatgcaacccatgaacgtaaaatgatgctggataatcatgccctgtacgataaaacgaaacgcatcttcctgaaagccgaaagcgaagaagaaatttttgcacatctgggccttgattacattgaaccgtgggaacgcaatgca

SEQ ID NO: 98 - DNA, 1167 bp, synthetic construct
  source 1..1167: mol_type = other DNA
atgggtcatcagctggttgttcgtaccgattatagcgcaaccccgaatccgggttttcagaaaacaccgcctctggcagttaaaaagattagccagtatgcatgtcagcgtcgtaccacactgaataactataaccatatctttaccgacgcctttgaaattctggcagaaaattcagaatttcgcgagaacgaagttagctatgttacctttatgcgtgcagcaagcgttctgaaaagcctgccgtttaccattattagcatgaaagataccgaaggtattccgtgtctgggtgataaagtgaaatgcatcattgaagagatcatcgaagatggtgaaagcagcgaagttaaagcagttctgaatgatgaacgttaccagagcttcaaactgtttaccagcgtttttggtgttggcctgaaaaccagcgaaaaatggtttcgtatgggttttcgtagcctgagcaaaattcgtagcgataaaaccctgaaattcaccaaaatgcagaaagccggtttcctgtattatgaagatctggttagctgcgttacccgtgccgaagccgaagcagttggtgttctggttaaagaagcagtttgggcatttctgccggatgcatttgttaccatgaccggtggttttcgtcgtggtaagaaaattggtcatgatgtggattttctgattaccagtccgggtagcgcagaagatgaagaacagctgctgccgaaagttattaatctgtgggaaaagaaaggtctgctgctgtattacgatctggttgaaagcaccttcgagaaattcaaactgccgagccgtcaggttgataccctggatcactttcagaaatgttttcttatcctgaagctgcatcatcagcgtgttgatagcagcaaaagcaatcagcaagaaggtaaaacctggaaagcaattcgtgttgatctggtgatgtgtccgtatgaacgtcgtgcatttgcactgttaggttggaccggtagtcgtcagtttgaacgtgatattcgtcgttatgcaacccatgaacgtaaaatgatgctggataatcatgccctgtacgataaaacgaaacgcgtgttcctgaaagccgaaagcgaagaagaaatttttgcacatctgggccttgattacattgaaccgtgggaacgtaatgca

SEQ ID NO: 99 - DNA, 1167 bp, synthetic construct
  source 1..1167: mol_type = other DNA
atgggtcatcagctggttgttcgtaccgattatagcgcaaccccgaatccgggttttcagaaaacaccgcctctggcagttaaaaagattagccagtatgcatgtcagcgtaaaaccacactgaataactgcaaccatatctttaccgatgcctttgaaattctggccgaaaactatgaatttcgcgagaatgaagttagctacgtgacctttatgcgtgcagcaagcgttctgaaaagcctgccgtttaccattattagcatgaaagataccgaaggtattccgtgtctgggtgataaagtgaaatgcatcattgaagagatcatcgaagatggtgaaagcagcgaagttaaagcagttctgaatgatgaacgttaccagagcttcaaactgtttaccagcgtttttggtgttggcctgaaaaccagcgaaaaatggtttcgtatgggttttcgtagcctgagcaaaattcgtagcgataaaaccctgaaatttacccgtatgcagaaagcgggttttctgtattatgaagatctggttagctgtgttacccgtgccgaagccgaagcagttggtgttctggttaaagaagcagtttgggcatttctgccggatgcatttgttaccatgaccggtggttttcgtcgtggtaagaaaattggtcatgatgtggattttctgattaccagtccgggtagcgcagaagatgaagaacagctgctgccgaaagttattaatctgtgggaaaagaaaggtctgctgctgtattacgatctggttgaaagcaccttcgagaaattcaaactgccgagccgtaaagttgatgcactggatcactttcagaaatgttttcttatcctgaagctgcatcatcagcgtgttgatagcggtaaaagcaatcagcaagaaggtaaaacctggaaagcaattcgtgttgatctggtgatgtgtccgtatgaaaatcgtgcatttgcactgttaggttggaccggtagccgtcagtttgaacgtgatattcgtcgttatgcaacccatgaacgtaaaatgatgctggataatcatgccctgtacgataaaacgaaacgcatcttcctgaaagccgaaagcgaagaagaaatttttgcacatctgggccttgattacattgaaccgtgggaacgtaatgca

SEQ ID NO: 100 - protein, 20 aa, synthetic construct
MGSSHHHHHHSSGENLYFQS